European Patent Specification EP 4 544 037 B1, published January 21, 2026. Title: CRISPR-Cas9 basierte Linearisierung von Plasmid DNA-Templaten. Applicant: Wacker Chemie AG. Application EP CO12114. The sequence listing filed with the application follows.

SEQUENCE LISTING (55 sequences)

SEQ ID NO: 1 - RNA, 101 nt, synthetic construct
  source 1..101: mol_type = other RNA
gaaaaaaaaaaaaaaaaagtcgttttagagctagaaatagcaagttaaaataaggctagtccgttatcaacttgaaaaagtggcaccgagtcggtgctttt

SEQ ID NO: 2 - protein, 1368 aa, Streptococcus pyogenes [sequence omitted]

SEQ ID NO: 3 - protein, 1053 aa, Staphylococcus aureus
MKRNYILGLDIGITSVGYGIIDYETRDVIDAGVRLFKEANVENNEGRRSKRGARRLKRRRRHRIQRVKKLLFDYNLLTDHSELSGINPYEARVKGLSQKLSEEEFSAALLHLAKRRGVHNVNEVEEDTGNELSTKEQISRNSKALEEKYVAELQLERLKKDGEVRGSINRFKTSDYVKEAKQLLKVQKAYHQLDQSFIDTYIDLLETRRTYYEGPGEGSPFGWKDIKEWYEMLMGHCTYFPEELRSVKYAYNADLYNALNDLNNLVITRDENEKLEYYEKFQIIENVFKQKKKPTLKQIAKEILVNEEDIKGYRVTSTGKPEFTNLKVYHDIKDITARKEIIENAELLDQIAKILTIYQSSEDIQEELTNLNSELTQEEIEQISNLKGYTGTHNLSLKAINLILDELWHTNDNQIAIFNRLKLVPKKVDLSQQKEIPTTLVDDFILSPVVKRSFIQSIKVINAIIKKYGLPNDIIIELAREKNSKDAQKMINEMQKRNRQTNERIEEIIRTTGKENAKYLIEKIKLHDMQEGKCLYSLEAIPLEDLLNNPFNYEVDHIIPRSVSFDNSFNNKVLVKQEENSKKGNRTPFQYLSSSDSKISYETFKKHILNLAKGKGRISKTKKEYLLEERDINRFSVQKDFINRNLVDTRYATRGLMNLLRSYFRVNNLDVKVKSINGGFTSFLRRKWKFKKERNKGYKHHAEDALIIANADFIFKEWKKLDKAKKVMENQMFEEKQAESMPEIETEQEYKEIFITPHQIKHIKDFKDYKYSHRVDKKPNRELINDTLYSTRKDDKGNTLIVNNLNGLYDKDNDKLKKLINKSPEKLLMYHHDPQTYQKLKLIMEQYGDEKNPLYKYYEETGNYLTKYSKKDNGPVIKKIKYYGNKLNAHLDITDDYPNSRNKVVKLSLKPYRFDVYLDNGVYKFVTVKNLDVIKKENYYEVNSKCYEEAKKLKKISNQAEFIASFYNNDLIKINGELYRVIGVNNDLLNRIEVNMIDITYREYLENMNDKRPPRIIKTIASKTQSIKKYSTDILGNLYEVKSKKHPQIIKKG

SEQ ID NO: 4 - protein, 1409 aa, Streptococcus thermophilus
MLFNKCIIISINLDFSNKEKCMTKPYSIGLDIGTNSVGWAVITDNYKVPSKKMKVLGNTSKKYIKKNLLGVLLFDSGITAEGRRLKRTARRRYTRRRNRILYLQEIFSTEMATLDDAFFQRLDDSFLVPDDKRDSKYPIFGNLVEEKVYHDEFPTIYHLRKYLADSTKKADLRLVYLALAHMIKYRGHFLIEGEFNSKNNDIQKNFQDFLDTYNAIFESDLSLENSKQLEEIVKDKISKLEKKDRILKLFPGEKNSGIFSEFLKLIVGNQADFRKCFNLDEKASLHFSKESYDEDLETLLGYIGDDYSDVFLKAKKLYDAILLSGFLTVTDNETEAPLSSAMIKRYNEHKEDLALLKEYIRNISLKTYNEVFKDDTKNGYAGYIDGKTNQEDFYVYLKNLLAEFEGADYFLEKIDREDFLRKQRTFDNGSIPYQIHLQEMRAILDKQAKFYPFLAKNKERIEKILTFRIPYYVGPLARGNSDFAWSIRKRNEKITPWNFEDVIDKESSAEAFINRMTSFDLYLPEEKVLPKHSLLYETFNVYNELTKVRFIAESMRDYQFLDSKQKKDIVRLYFKDKRKVTDKDIIEYLHAIYGYDGIELKGIEKQFNSSLSTYHDLLNIINDKEFLDDSSNEAIIEEIIHTLTIFEDREMIKQRLSKFENIFDKSVLKKLSRRHYTGWGKLSAKLINGIRDEKSGNTILDYLIDDGISNRNFMQLIHDDALSFKKKIQKAQIIGDEDKGNIKEVVKSLPGSPAIKKGILQSIKIVDELVKVMGGRKPESIVVEMARENQYTNQGKSNSQQRLKRLEKSLKELGSKILKENIPAKLSKIDNNALQNDRLYLYYLQNGKDMYTGDDLDIDRLSNYDIDHIIPQAFLKDNSIDNKVLVSSASNRGKSDDFPSLEVVKKRKTFWYQLLKSKLISQRKFDNLTKAERGGLLPEDKAGFIQRQLVETRQITKHVARLLDEKFNNKKDENNRAVRTVKIITLKSTLVSQFRKDFELYKVREINDFHHAHDAYLNAVIASALLKKYPKLEPEFVYGDYPKYNSFRERKSATEKVYFYSNIMNIFKKSISLADGRVIERPLIEVNEETGESVWNKESDLATVRRVLSYPQVNVVKKVEEQNHGLDRGKPKGLFNANLSSKPKPNSNENLVGAKEYLDPKKYGGYAGISNSFAVLVKGTIEKGAKKKITNVLEFQGISILDRINYRKDKLNFLLEKGYKDIELIIELPKYSLFELSDGSRRMLASILSTNNKRGEIHKGNQIFLSQKFVKLLYHAKRISNTINENHRKYVENHKKEFEELFYYILEFNENYVGAKKNGKLLNSAFQSWQNHSIDELCSSFIGPTGSERKGLFELTSRGSAADFEFLGVKIPRYRDYTPSSLLKDATLIHQSVTGLYETRIDLAKLGEG

SEQ ID NO: 5 - DNA, 5545 bp, synthetic construct
  source 1..5545: mol_type = other DNA
ttgacaattaatcatcggctcgtataatgtgtggaattgtgagcggataacaatttcacacaggaaacagaattctaaggaggaaattatatggctagcaaaggagaagaacttttcactggagttgtcccaattcttgttgaattagatggtgatgttaatgggcacaaattttctgtcagtggagagggtgaaggtgatgctacatacggaaagcttacccttaaatttatttgcactactggaaaactacctgttccatggccaacacttgtcactactttctcttatggtgttcaatgcttttcccgttatccggatcatatgaaacggcatgactttttcaagagtgccatgcccgaaggttatgtacaggaacgcactatatctttcaaagatgacgggaactacaagacgcgtgctgaagtcaagtttgaaggtgatacccttgttaatcgtatcgagttaaaaggtattgattttaaagaagatggaaacattctcggacacaaactcgagtacaactataactcacacaatgtatacatcacggcagacaaacaaaagaatggaatcaaagctaacttcaaaattcgccacaacattgaagatggatccgttcaactagcagaccattatcaacaaaatactccaattggcgatggccctgtccttttaccagacaaccattacctgtcgacacaatctgccctttcgaaagatcccaacgaaaagcgtgaccacatggtccttcttgagtttgtaactgctgctgggattacacatggcatggatgagctctacaaataatctagaagcttggctgttttggcggatgagagaagattttcagcctgatacagattaaatcagaacgcagaagcggtctgataaaacagaatttgcctggcggcagtagcgcggtggtcccacctgaccccatgccgaactcagaagtgaaacgccgtagcgccgatggtagtgtggggtctccccatgcgagagtagggaactgccaggcatcaaataaaacgaaaggctcagtcgaaagactgggcctttcgttttatctgttgtttgtcggtgaacgctctcctgagtaggacaaatccgccgggagcggatttgaacgttgcgaagcaacggcccggagggtggcgggcaggacgcccgccataaactgccaggcatcaaattaagcagaaggccatcctgacggatggcctttttgcgtttctacaaactcttttgtttatttttctaaatacattcaaatatgtatccgctcatgagacaataaccctgataaatgcttcaataatattgaaaaaggaagagtatgagtattcaacatttccgtgtcgcccttattcccttttttgcggcattttgccttcctgtttttgctcacccagaaacgctggtgaaagtaaaagatgctgaagatcagttgggtgcacgagtgggttacatcgaactggatctcaacagcggtaagatccttgagagttttcgccccgaagaacgttttccaatgatgagcacttttgcggccgcatatgagctctccggaagatctctcgaggtcgacgtacgtgcccatggatgcatttaattaattcgaagttaacttaagcttgtacactagtaaagttctgctatgtggcgcggtattatcccgtgttgacgccgggcaagagcaactcggtcgccgcatacactattctcagaatgacttggttgagtccatggcggccgccttcatgtggcaggagaaaaaaggctgcaccggtgcgtcagcagaatatgtgatacaggatatattccgcttcctcgctcactgactcgctacgctcggtcgttcgactgcggcgagcggaaatggcttacgaacggggcggagatttcctggaagatgccaggaagatacttaacagggaagtgagagggccgcggcaaagccgtttttccataggctccgcccccctgacaagcatcacgaaatctgacgctcaaatcagtggtggcgaaacccgacaggactataaagataccaggcgtttccccctggcggctccctcgtgcgctctcctgttcctgcctttcggtttaccggtgtcattccgctgttatggccgcgtttgtctcattccacgcctgacactcagttccgggtaggcagttcgctccaagctggactgtatgcacgaaccccccgttcagtccgaccgctgcgccttatccggtaactatcgtcttgagtccaacccggaaagacatgcaaaagcaccactggcagcagccactggtaattgatttagaggagttagtcttgaagtcatgcgccggttaaggctaaactgaaaggacaagttttggtgactgcgctcctccaagccagttacctcggttcaaagagttggtagctcagagaaccttcgaaaaaccgccctgcaaggcggttttttcgttttcagagcaagagattacgcgcagaccaaaacgatctcaagaagatcatcttattaatcagataaaatatttctagctagatttcagtgcaatttatctcttcaaatgtagcacctgaagtcagccccatacgatataagttgtaattctcatgtttgacagcttatcatcgataagctccaggacccaacgctgcccgagatgcgccgcgtgcggctgctggagatggcggacgcgatggatatgttctgccaagggttggtttgcgcattcacagttctccgcaagaattgattggctccaattcttggagtggtgaatccgttagcgaggtgccgccggcttccattcaggtcgaggtggcccggctccatgcaccgcgacgcaacgcggggaggcagacaaggtatagggcggcgcctacaatccatgccaacccgttccatgtgctcgccgaggcggcataaatcgccgtgacgatcagcggtccaatgatcgaagttaggctggtaagagccgcgagcgatccttgaagctgtccctgatggtcgtcatctacctgcctggacagcatggcctgcaacgcgggcatcccgatgccgccggaagcgagaagaatcataatggggaaggccatccagcctcgcgtcgcgaacgccagcaagacgtagcccagcgcgtcggccgccatgccggcgataatggcctgcttctcgccgaaacgtttggtggcgggaccagtgacgaaggcttgagcgagggcgtgcaagattccgaataccgcaagcgacaggccgatcatcgtcgcgctccagcgaaagcggtcctcgccgaaaatgacccagagcgctgccggcacctgtcctacgagttgcatgataaagaagacagtcataagtgcggcgacgatagtcatgccccgcgcccaccggaaggagctgactgggttgaaggctctcaagggcatcggtcgacgctctcccttatgcgactcctgcattaggaagcagcccagtagtaggttgaggccgttgagcaccgccgccgcaaggaatggtgcatgcaaggagatggcgcccaacagtcccccggccacggggcctgccaccatacccacgccgaaacaagcgctcatgagcccgaagtggcgagcccgatcttccccatcggtgatgtcggcgatataggcgccagcaaccgcacctgtggcgccggtgatgccggccacgatgcgtccggcgtagaggatccacaggacgggtgtggtcgccatgatcgcgtagtcgatagtggctccaagtagcgaagcgagcaggactgggcggcggccaaagcggtcggacagtgctccgagaacgggtgcgcatagaaattgcatcaacgcatatagcgctagcagcacgccatagtgactggcgatgctgtcggaatggacgatatcccgcaagaggcccggcagtaccggcataaccaagcctatgcctacagcatccagggtgacggtgccgaggatgacgatgagcgcattgttagatttcatacacggtgcctgactgcgttagcaatttaactgtgataaactaccgcattaaagcttatcgatgataagctgtcaaacatggcctgtcgcttgcggtattcggaatcttgcacgccctcgctcaagccttcgtcactggtcccgccaccaaacgtttcggcgagaagcaggccattatcgccggcatggcggccgacgcgctgggagaggcggtttgcgtattgggcgccagggtggtttttcttttcaccagtgagacgggcaacagctgattgcccttcaccgcctggccctgagagagttgcagcaagcggtccacgctggtttgccccagcaggcgaaaatcctgtttgatggtggttaacggcgggatataacatgagctgtcttcggtatcgtcgtatcccactaccgagatatccgcaccaacgcgcagcccggactcggtaatggcgcgcattgcgcccagcgccatctgatcgttggcaaccagcatcgcagtgggaacgatgccctcattcagcatttgcatggtttgttgaaaaccggacatggcactccagtcgccttcccgttccgctatcggctgaatttgattgcgagtgagatatttatgccagccagccagacgcagacgcgccgagacagaacttaatgggcccgctaacagcgcgatttgctggtgacccaatgcgaccagatgctccacgcccagtcgcgtaccgtcttcatgggagaaaataatactgttgatgggtgtctggtcagagacatcaagaaataacgccggaacattagtgcaggcagcttccacagcaatggcatcctggtcatccagcggatagttaatgatcagcccactgacgcgttgcgcgagaagattgtgcaccgccgctttacaggcttcgacgccgcttcgttctaccatcgacaccaccacgctggcacccagttgatcggcgcgagatttaatcgccgcgacaatttgcgacggcgcgtgcagggccagactggaggtggcaacgccaatcagcaacgactgtttgcccgccagttgttgtgccacgcggttgggaatgtaattcagctccgccatcgccgcttccactttttcccgcgttttcgcagaaacgtggctggcctggttcaccacgcgggaaacggtctgataagagacaccggcatactctgcgacatcgtataacgttactggtttcacattcaccaccctgaattgactctcttccgggcgctatcatgccataccgcgaaaggttttgcaccattcgatggtgtcaacgtaaatgcatgccgcttcgccttcgcgcgcgaattgcaagctgatccgggcttatcgactgcacggtgcaccaatgcttctggcgtcaggcagccatcggaagctgtggtatggctgtgcaggtcgtaaatcactgcataattcgtgtcgctcaaggcgcactcccgttctggataatgttttttgcgccgacatcataacggttctggcaaatattgtggaattgtgagcgg

SEQ ID NO: 6 - DNA, 1452 bp, synthetic construct
  source 1..1452: mol_type = other DNA
tgaaattgttatccgctcacaattccacacattatacgagccgatgattaattgtcaaccgctcacaattccacaatatttgccagaaccgttatgatgtcggcgcaaaaaacattatccagaacgggagtgcgccttgagcgacacgaattatgcagtgatttacgacctgcacagccataccacagcttccgatggctgcctgacgccagaagcattggtgcaccgtgcagtcgataagcccggatcagcttgcaattcgcgcgcgaaggcgaagcggcatgcatttacgttgacaccatcgaatggtgcaaaacctttcgcggtatggcatgatagcgcccggaagagagtcaattcagggtggtgaatgtgaaaccagtaacgttatacgatgtcgcagagtatgccggtgtctcttatcagaccgtttcccgcgtggtgaaccaggccagccacgtttctgcgaaaacgcgggaaaaagtggaagcggcgatggcggagctgaattacattcccaaccgcgtggcacaacaactggcgggcaaacagtcgttgctgattggcgttgccacctccagtctggccctgcacgcgccgtcgcaaattgtcgcggcgattaaatctcgcgccgatcaactgggtgccagcgtggtggtgtcgatggtagaacgaagcggcgtcgaagcctgtaaagcggcggtgcacaatcttctcgcgcaacgcgtcagtgggctgatcattaactatccgctggatgaccaggatgccattgctgtggaagctgcctgcactaatgttccggcgttatttcttgatgtctctgaccagacacccatcaacagtattattttctcccatgaagacggtacgcgactgggcgtggagcatctggtcgcattgggtcaccagcaaatcgcgctgttagcgggcccattaagttctgtctcggcgcgtctgcgtctggctggctggcataaatatctcactcgcaatcaaattcagccgatagcggaacgggaaggcgactggagtgccatgtccggttttcaacaaaccatgcaaatgctgaatgagggcatcgttcccactgcgatgctggttgccaacgatcagatggcgctgggcgcaatgcgcgccattaccgagtccgggctgcgcgttggtgcggatatctcggtagtgggatacgacgataccgaagacagctcatgttatatcccgccgttaaccaccatcaaacaggattttcgcctgctggggcaaaccagcgtggaccgcttgctgcaactctctcagggccaggcggtgaagggcaatcagctgttgcccgtctcactggtgaaaagaaaaaccaccctggcgcccaatacgcaaaccgcctctccccgcgcgttggccgattcattaatgcagctggcacgacaggtttcccgactggaaagcgggcag

SEQ ID NO: 7 - DNA, 1386 bp, synthetic construct
  source 1..1386: mol_type = other DNA
agaggcggtttgcgtattgggcgccagggtggtttttcttttcaccagtgagacgggcaacagctgattgcccttcaccgcctggccctgagagagttgcagcaagcggtccacgctggtttgccccagcaggcgaaaatcctgtttgatggtggttaacggcgggatataacatgagctgtcttcggtatcgtcgtatcccactaccgagatatccgcaccaacgcgcagcccggactcggtaatggcgcgcattgcgcccagcgccatctgatcgttggcaaccagcatcgcagtgggaacgatgccctcattcagcatttgcatggtttgttgaaaaccggacatggcactccagtcgccttcccgttccgctatcggctgaatttgattgcgagtgagatatttatgccagccagccagacgcagacgcgccgagacagaacttaatgggcccgctaacagcgcgatttgctggtgacccaatgcgaccagatgctccacgcccagtcgcgtaccgtcttcatgggagaaaataatactgttgatgggtgtctggtcagagacatcaagaaataacgccggaacattagtgcaggcagcttccacagcaatggcatcctggtcatccagcggatagttaatgatcagcccactgacgcgttgcgcgagaagattgtgcaccgccgctttacaggcttcgacgccgcttcgttctaccatcgacaccaccacgctggcacccagttgatcggcgcgagatttaatcgccgcgacaatttgcgacggcgcgtgcagggccagactggaggtggcaacgccaatcagcaacgactgtttgcccgccagttgttgtgccacgcggttgggaatgtaattcagctccgccatcgccgcttccactttttcccgcgttttcgcagaaacgtggctggcctggttcaccacgcgggaaacggtctgataagagacaccggcatactctgcgacatcgtataacgttactggtttcacattcaccaccctgaattgactctcttccgggcgctatcatgccataccgcgaaaggttttgcaccattcgatggtgtcaacgtaaatgcatgccgcttcgccttcgcgcgcgaattgcaagctgatccgggcttatcgactgcacggtgcaccaatgcttctggcgtcaggcagccatcggaagctgtggtatggctgtgcaggtcgtaaatcactgcataattcgtgtcgctcaaggcgcactcccgttctggataatgttttttgcgccgacatcataacggttctggcaaatattgtggaattgtgagcggttgacaattaatcatcggctcgtataatgtgtggaattgtgagcggataacaatttca

SEQ ID NO: 8 - DNA, 67 bp, synthetic construct
  source 1..67: mol_type = other DNA
gaatccgaattctaatacgactcactatagggataaaggaggtaaataatggctagcaaaggagaag

SEQ ID NO: 9 - DNA, 100 bp, synthetic construct
  source 1..100: mol_type = other DNA
ttgcactctagagccgacttttttttttttttttttttttttttttttttttttttttttttttttttttttttttttttatttgtagagctcatccatg

SEQ ID NO: 10 - DNA, 846 bp, synthetic construct
  source 1..846: mol_type = other DNA
gaatccgaattctaatacgactcactatagggataaaggaggtaaataatggctagcaaaggagaagaacttttcactggagttgtcccaattcttgttgaattagatggtgatgttaatgggcacaaattttctgtcagtggagagggtgaaggtgatgctacatacggaaagcttacccttaaatttatttgcactactggaaaactacctgttccatggccaacacttgtcactactttctcttatggtgttcaatgcttttcccgttatccggatcatatgaaacggcatgactttttcaagagtgccatgcccgaaggttatgtacaggaacgcactatatctttcaaagatgacgggaactacaagacgcgtgctgaagtcaagtttgaaggtgatacccttgttaatcgtatcgagttaaaaggtattgattttaaagaagatggaaacattctcggacacaaactcgagtacaactataactcacacaatgtatacatcacggcagacaaacaaaagaatggaatcaaagctaacttcaaaattcgccacaacattgaagatggatccgttcaactagcagaccattatcaacaaaatactccaattggcgatggccctgtccttttaccagacaaccattacctgtcgacacaatctgccctttcgaaagatcccaacgaaaagcgtgaccacatggtccttcttgagtttgtaactgctgctgggattacacatggcatggatgagctctacaaataaaaaaaaaaaaaaaaaaaaaaaaaaaaaaaaaaaaaaaaaaaaaaaaaaaaaaaaaaaaaagtcggctctagagtgcaa

SEQ ID NO: 11 - DNA, 3487 bp, synthetic construct
  source 1..3487: mol_type = other DNA
gacgaaagggcctcgtgatacgcctatttttataggttaatgtcatgataataatggtttcttagacgtcaggtggcacttttcggggaaatgtgcgcggaacccctatttgtttatttttctaaatacattcaaatatgtatccgctcatgagacaataaccctgataaatgcttcaataatattgaaaaaggaagagtatgagtattcaacatttccgtgtcgcccttattcccttttttgcggcattttgccttcctgtttttgctcacccagaaacgctggtgaaagtaaaagatgctgaagatcagttgggtgcacgagtgggttacatcgaactggatctcaacagcggtaagatccttgagagttttcgccccgaagaacgttttccaatgatgagcacttttaaagttctgctatgtggcgcggtattatcccgtattgacgccgggcaagagcaactcggtcgccgcatacactattctcagaatgacttggttgagtactcaccagtcacagaaaagcatcttacggatggcatgacagtaagagaattatgcagtgctgccataaccatgagtgataacactgcggccaacttacttctgacaacgatcggaggaccgaaggagctaaccgcttttttgcacaacatgggggatcatgtaactcgccttgatcgttgggaaccggagctgaatgaagccataccaaacgacgagcgtgacaccacgatgcctgtagcaatggcaacaacgttgcgcaaactattaactggcgaactacttactctagcttcccggcaacaattaatagactggatggaggcggataaagttgcaggaccacttctgcgctcggcccttccggctggctggtttattgctgataaatctggagccggtgagcgtgggtctcgcggtatcattgcagcactggggccagatggtaagccctcccgtatcgtagttatctacacgacggggagtcaggcaactatggatgaacgaaatagacagatcgctgagataggtgcctcactgattaagcattggtaactgtcagaccaagtttactcatatatactttagattgatttaaaacttcatttttaatttaaaaggatctaggtgaagatcctttttgataatctcatgaccaaaatcccttaacgtgagttttcgttccactgagcgtcagaccccgtagaaaagatcaaaggatcttcttgagatcctttttttctgcgcgtaatctgctgcttgcaaacaaaaaaaccaccgctaccagcggtggtttgtttgccggatcaagagctaccaactctttttccgaaggtaactggcttcagcagagcgcagataccaaatactgttcttctagtgtagccgtagttaggccaccacttcaagaactctgtagcaccgcctacatacctcgctctgctaatcctgttaccagtggctgctgccagtggcgataagtcgtgtcttaccgggttggactcaagacgatagttaccggataaggcgcagcggtcgggctgaacggggggttcgtgcacacagcccagcttggagcgaacgacctacaccgaactgagatacctacagcgtgagctatgagaaagcgccacgcttcccgaagggagaaaggcggacaggtatccggtaagcggcagggtcggaacaggagagcgcacgagggagcttccagggggaaacgcctggtatctttatagtcctgtcgggtttcgccacctctgacttgagcgtcgatttttgtgatgctcgtcaggggggcggagcctatggaaaaacgccagcaacgcggcctttttacggttcctggccttttgctggccttttgctcacatgttctttcctgcgttatcccctgattctgtggataaccgtattaccgcctttgagtgagctgataccgctcgccgcagccgaacgaccgagcgcagcgagtcagtgagcgaggaagcggaagagcgcccaatacgcaaaccgcctctccccgcgcgttggccgattcattaatgcagctggcacgacaggtttcccgactggaaagcgggcagtgagcgcaacgcaattaatgtgagttagctcactcattaggcaccccaggctttacactttatgcttccggctcgtatgttgtgtggaattgtgagcggataacaatttcacacaggaaacagctatgaccatgattacgccgaattctaatacgactcactatagggataaaggaggtaaataatggctagcaaaggagaagaacttttcactggagttgtcccaattcttgttgaattagatggtgatgttaatgggcacaaattttctgtcagtggagagggtgaaggtgatgctacatacggaaagcttacccttaaatttatttgcactactggaaaactacctgttccatggccaacacttgtcactactttctcttatggtgttcaatgcttttcccgttatccggatcatatgaaacggcatgactttttcaagagtgccatgcccgaaggttatgtacaggaacgcactatatctttcaaagatgacgggaactacaagacgcgtgctgaagtcaagtttgaaggtgatacccttgttaatcgtatcgagttaaaaggtattgattttaaagaagatggaaacattctcggacacaaactcgagtacaactataactcacacaatgtatacatcacggcagacaaacaaaagaatggaatcaaagctaacttcaaaattcgccacaacattgaagatggatccgttcaactagcagaccattatcaacaaaatactccaattggcgatggccctgtccttttaccagacaaccattacctgtcgacacaatctgccctttcgaaagatcccaacgaaaagcgtgaccacatggtccttcttgagtttgtaactgctgctgggattacacatggcatggatgagctctacaaataaaaaaaaaaaaaaaaaaaaaaaaaaaaaaaaaaaaaaaaaaaaaaaaaaaaaaaaaaaaaagtcggctctagagtcgacctgcaggcatgcaagcttactggccgtcgttttacaacgtcgtgactgggaaaaccctggcgttacccaacttaatcgccttgcagcacatccccctttcgccagctggcgtaatagcgaagaggcccgcaccgatcgcccttcccaacagttgcgcagcctgaatggcgaatggcgcctgatgcggtattttctccttacgcatctgtgcggtatttcacaccgcatatggtgcactctcagtacaatctgctctgatgccgcatagttaagccagccccgacacccgccaacacccgctgacgcgccctgacgggcttgtctgctcccggcatccgcttacagacaagctgtgaccgtctccgggagctgcatgtgtcagaggttttcaccgtcatcaccgaaacgcgcga

SEQ ID NO: 12 - DNA, 121 bp, synthetic construct
  source 1..121: mol_type = other DNA
aaaagcaccgactcggtgccactttttcaagttgataacggactagccttattttaacttgctatttctagctctaaaacgactttttttttttttttttctatagtgagtcgtattagaa

SEQ ID NO: 13 - DNA, 21 bp, synthetic construct
  source 1..21: mol_type = other DNA
ttctaatacgactcactatag

SEQ ID NO: 14 - DNA, 3489 bp, synthetic construct
  source 1..3489: mol_type = other DNA
gacgaaagggcctcgtgatacgcctatttttataggttaatgtcatgataataatggtttcttagacgtcaggtggcacttttcggggaaatgtgcgcggaacccctatttgtttatttttctaaatacattcaaatatgtatccgctcatgagacaataaccctgataaatgcttcaataatattgaaaaaggaagagtatgagtattcaacatttccgtgtcgcccttattcccttttttgcggcattttgccttcctgtttttgctcacccagaaacgctggtgaaagtaaaagatgctgaagatcagttgggtgcacgagtgggttacatcgaactggatctcaacagcggtaagatccttgagagttttcgccccgaagaacgttttccaatgatgagcacttttaaagttctgctatgtggcgcggtattatcccgtattgacgccgggcaagagcaactcggtcgccgcatacactattctcagaatgacttggttgagtactcaccagtcacagaaaagcatcttacggatggcatgacagtaagagaattatgcagtgctgccataaccatgagtgataacactgcggccaacttacttctgacaacgatcggaggaccgaaggagctaaccgcttttttgcacaacatgggggatcatgtaactcgccttgatcgttgggaaccggagctgaatgaagccataccaaacgacgagcgtgacaccacgatgcctgtagcaatggcaacaacgttgcgcaaactattaactggcgaactacttactctagcttcccggcaacaattaatagactggatggaggcggataaagttgcaggaccacttctgcgctcggcccttccggctggctggtttattgctgataaatctggagccggtgagcgtgggtctcgcggtatcattgcagcactggggccagatggtaagccctcccgtatcgtagttatctacacgacggggagtcaggcaactatggatgaacgaaatagacagatcgctgagataggtgcctcactgattaagcattggtaactgtcagaccaagtttactcatatatactttagattgatttaaaacttcatttttaatttaaaaggatctaggtgaagatcctttttgataatctcatgaccaaaatcccttaacgtgagttttcgttccactgagcgtcagaccccgtagaaaagatcaaaggatcttcttgagatcctttttttctgcgcgtaatctgctgcttgcaaacaaaaaaaccaccgctaccagcggtggtttgtttgccggatcaagagctaccaactctttttccgaaggtaactggcttcagcagagcgcagataccaaatactgttcttctagtgtagccgtagttaggccaccacttcaagaactctgtagcaccgcctacatacctcgctctgctaatcctgttaccagtggctgctgccagtggcgataagtcgtgtcttaccgggttggactcaagacgatagttaccggataaggcgcagcggtcgggctgaacggggggttcgtgcacacagcccagcttggagcgaacgacctacaccgaactgagatacctacagcgtgagctatgagaaagcgccacgcttcccgaagggagaaaggcggacaggtatccggtaagcggcagggtcggaacaggagagcgcacgagggagcttccagggggaaacgcctggtatctttatagtcctgtcgggtttcgccacctctgacttgagcgtcgatttttgtgatgctcgtcaggggggcggagcctatggaaaaacgccagcaacgcggcctttttacggttcctggccttttgctggccttttgctcacatgttctttcctgcgttatcccctgattctgtggataaccgtattaccgcctttgagtgagctgataccgctcgccgcagccgaacgaccgagcgcagcgagtcagtgagcgaggaagcggaagagcgcccaatacgcaaaccgcctctccccgcgcgttggccgattcattaatgcagctggcacgacaggtttcccgactggaaagcgggcagtgagcgcaacgcaattaatgtgagttagctcactcattaggcaccccaggctttacactttatgcttccggctcgtatgttgtgtggaattgtgagcggataacaatttcacacaggaaacagctatgaccatgattacgccgaattctaatacgactcactatagggataaaggaggtaaataatggctagcaaaggagaagaacttttcactggagttgtcccaattcttgttgaattagatggtgatgttaatgggcacaaattttctgtcagtggagagggtgaaggtgatgctacatacggaaagcttacccttaaatttatttgcactactggaaaactacctgttccatggccaacacttgtcactactttctcttatggtgttcaatgcttttcccgttatccggatcatatgaaacggcatgactttttcaagagtgccatgcccgaaggttatgtacaggaacgcactatatctttcaaagatgacgggaactacaagacgcgtgctgaagtcaagtttgaaggtgatacccttgttaatcgtatcgagttaaaaggtattgattttaaagaagatggaaacattctcggacacaaactcgagtacaactataactcacacaatgtatacatcacggcagacaaacaaaagaatggaatcaaagctaacttcaaaattcgccacaacattgaagatggatccgttcaactagcagaccattatcaacaaaatactccaattggcgatggccctgtccttttaccagacaaccattacctgtcgacacaatctgccctttcgaaagatcccaacgaaaagcgtgaccacatggtccttcttgagtttgtaactgctgctgggattacacatggcatggatgagctctacaaataaaaaaaaaaaaaaaaaaaaaaaaaaaaaaaaaaaaaaaaaaaaaaaaaaaaaaaaaaaaaaaagtcttctctagagtcgacctgcaggcatgcaagcttactggccgtcgttttacaacgtcgtgactgggaaaaccctggcgttacccaacttaatcgccttgcagcacatccccctttcgccagctggcgtaatagcgaagaggcccgcaccgatcgcccttcccaacagttgcgcagcctgaatggcgaatggcgcctgatgcggtattttctccttacgcatctgtgcggtatttcacaccgcatatggtgcactctcagtacaatctgctctgatgccgcatagttaagccagccccgacacccgccaacacccgctgacgcgccctgacgggcttgtctgctcccggcatccgcttacagacaagctgtgaccgtctccgggagctgcatgtgtcagaggttttcaccgtcatcaccgaaacgcgcga

SEQ ID NO: 15 - DNA, 102 bp, synthetic construct
  source 1..102: mol_type = other DNA
ttgcactctagagaagacttttttttttttttttttttttttttttttttttttttttttttttttttttttttttttttttatttgtagagctcatccatg

SEQ ID NO: 16 - DNA, 828 bp, synthetic construct
  source 1..828: mol_type = other DNA
gaatccgaattctaatacgactcactatagggataaaggaggtaaataatggctagcaaaggagaagaacttttcactggagttgtcccaattcttgttgaattagatggtgatgttaatgggcacaaattttctgtcagtggagagggtgaaggtgatgctacatacggaaagcttacccttaaatttatttgcactactggaaaactacctgttccatggccaacacttgtcactactttctcttatggtgttcaatgcttttcccgttatccggatcatatgaaacggcatgactttttcaagagtgccatgcccgaaggttatgtacaggaacgcactatatctttcaaagatgacgggaactacaagacgcgtgctgaagtcaagtttgaaggtgatacccttgttaatcgtatcgagttaaaaggtattgattttaaagaagatggaaacattctcggacacaaactcgagtacaactataactcacacaatgtatacatcacggcagacaaacaaaagaatggaatcaaagctaacttcaaaattcgccacaacattgaagatggatccgttcaactagcagaccattatcaacaaaatactccaattggcgatggccctgtccttttaccagacaaccattacctgtcgacacaatctgccctttcgaaagatcccaacgaaaagcgtgaccacatggtccttcttgagtttgtaactgctgctgggattacacatggcatggatgagctctacaaataaaaaaaaaaaaaaaaaaaaaaaaaaaaaaaaaaaaaaaaaaaaaaaaaaaaaaaaaaaaaa

SEQ ID NO: 17 - DNA, 67 bp, synthetic construct; identical to SEQ ID NO: 8
  source 1..67: mol_type = other DNA

SEQ ID NO: 18 - DNA, 82 bp, synthetic construct
  source 1..82: mol_type = other DNA
ttttttttttttttttttttttttttttttttttttttttttttttttttttttttttttttatttgtagagctcatccatg

SEQ ID NO: 19 - DNA, 18 bp, synthetic construct
  source 1..18: mol_type = other DNA
tgtgcggcattcttatta

SEQ ID NO: 20 - DNA, 21 bp, synthetic construct
  source 1..21: mol_type = other DNA
catggcatggatgagctctac

SEQ ID NO: 21 - DNA, 18 bp, synthetic construct
  source 1..18: mol_type = other DNA
taataagaatgccgcaca

SEQ ID NO: 22 - DNA, 46 bp, synthetic construct
  source 1..46: mol_type = other DNA
atccacgaattcaggaggcaaaaatggacaaaaaatacagcattgg

SEQ ID NO: 23 - DNA, 129 bp, synthetic construct
  source 1..129: mol_type = other DNA
atccactctagaatccacggtaccatccacatccacatccacatccacacagggataaaaaaagcagcactgtaatcagtgctgctttgtcgtttttttcatcatcatcaatcaccacctaactggctc

SEQ ID NO: 24 - DNA, 10884 bp, synthetic construct
  source 1..10884: mol_type = other DNA
catggggtttgcagtcagagtagaatagaagtatcaaaaaaagcaccgactcggtgccactttttcaagttgataacggactagccttattttaacttgctatgctgttttgaatggttccaacaagattattttataacttttataacaaataatcaaggagaaattcaaagaaatttatcagccataaaacaatacttaatactatagaatgataacaaaataaactactttttaaaagaattttgtgttataatctatttattattaagtattgggtaatattttttgaagagatattttgaaaaagaaaaattaaagcatattaaactaatttcggaggtcattaaaactattattgaaatcatcaaactcattatggatttaatttaaactttttattttaggaggcaaaaatggacaaaaaatacagcattggtctggatattggcaccaatagcgttggttgggcagttattaccgatgaatataaagttccgagcaaaaaattcaaggtgctgggtaataccgatcgccatagcattaaaaagaatctgattggtgcactgctgttcgatagcggtgaaaccgcagaagcaacccgtctgaaacgtaccgcacgtcgtcgttatacccgtcgtaaaaatcgtatttgctatctgcaagagatctttagcaacgaaatggccaaagtggatgatagcttttttcatcgtctggaagaatcctttctggtggaagaagataaaaaacacgaacgccatccgatttttggcaacattgttgatgaagtggcctaccatgaaaaatatccgaccatttatcatctgcgcaaaaaactggttgatagcaccgataaagccgatctgcgtctgatttatctggcactggcacatatgatcaaatttcgtggtcattttctgatcgaaggtgatctgaatccggataatagtgatgtggataaactgttcattcagctggtgcagacctataatcagctgtttgaagaaaatccgattaatgccagcggtgttgatgcaaaagcaattctgagcgcacgtctgagcaaaagccgtcgcctggaaaacctgattgcacagctgcctggtgaaaaaaagaatggtctgtttggtaatctgatcgcactgagcctgggtctgaccccgaactttaaatcaaattttgatctggccgaagatgccaaactgcagctgagcaaagatacctatgatgatgatctggataatctgctggcacagattggtgatcagtatgcagacctgtttctggcagcgaaaaatctgagtgatgcaattctgctgagcgatattctgcgtgttaataccgaaattaccaaagcaccgctgagcgcaagtatgattaaacgttatgatgaacatcaccaggatctgaccctgctgaaagcactggttcgtcagcagctgccggaaaagtataaagaaatctttttcgaccagagcaagaatggctatgccggttatattgatggtggtgcaagccaagaagagttctacaaattcattaaaccgatcctggaaaagatggatggcaccgaagaactgctggttaaactgaatcgtgaagatctgctgcgtaaacagcgtacctttgataatggtagcattccgcatcagattcatctgggtgaactgcatgccattctgcgtcgtcaagaagatttttatccgttcctgaaagataaccgcgagaaaatcgaaaaaattctgacctttcgcatcccgtattatgtgggtccgctggcacgtggtaatagccgttttgcatggatgacccgtaaaagcgaagaaaccattacaccgtggaatttcgaagaggttgttgataaaggtgcaagcgcacagagctttattgaacgtatgaccaacttcgataaaaacctgccgaatgaaaaagttctgccgaaacatagcctgctgtatgaatatttcaccgtgtataatgagctgaccaaagtgaaatatgtgaccgaaggtatgcgtaaaccggcatttctgagcggtgaacagaaaaaagcgattgttgatctgctgtttaaaaccaatcgtaaggttaccgttaagcagctgaaagaggattatttcaaaaaaatcgagtgctttgatagcgtcgaaattagcggtgtggaagatcgttttaatgcaagcctgggcacctatcacgatctgctgaaaatcattaaagataaagattttctggacaacgaagagaacgaggacattctggaagatattgttctgacactgaccctgtttgaggatcgtgaaatgattgaagaacgcctgaaaacatatgcccacctgttcgatgataaagtgatgaaacaactgaaacgccgtcgctataccggttggggtcgtctgagccgtaaactgattaatggtattcgtgataaacagagcggcaaaaccattctggattttctgaaaagtgatggctttgccaatcgcaattttatgcagctgattcatgatgatagcctgacctttaaagaggatattcagaaagcacaggttagcggtcagggtgatagtctgcatgaacatattgcaaatctggcaggtagtccggcaatcaaaaaaggtattctgcagaccgttaaagtggttgatgaactggttaaagttatgggtcgtcataaaccggaaaacatcgtgattgaaatggcacgtgaaaatcagaccacacagaaaggccagaaaaatagccgtgaacgcatgaaacgtattgaagaaggtattaaagaactgggcagccagattctgaaagaacatccggttgaaaatacccagctgcagaacgaaaaactgtatctgtattacctgcagaatggtcgtgacatgtatgttgatcaagaactggatattaatcgcctgagcgattatgatgtcgatcatattgttccgcagtcctttcttaaagatgatagcattgacaacaaagtgctgacccgtagcgacaaaaatcgtggtaaaagtgataatgtgccgagcgaagaggtggttaaaaagatgaaaaactattggcgtcaactgctgaacgccaaactgatcacacagcgcaaatttgataatctgacaaaagcagaacgtggtggtctgagcgagctggataaagcaggttttatcaaacgtcagctggttgaaacccgtcagatcacaaaacatgttgcacagattctggatagccgcatgaataccaaatatgacgaaaacgataaactgatccgcgaggttaaagtgattaccctgaaaagcaaactggtgagcgattttcgtaaagacttccagttttacaaagtgcgcgaaatcaacaattatcatcacgcacatgatgcctatctgaatgcagttgttggcaccgcactgattaagaaatatcctaaactggaaagcgagttcgtgtatggcgattataaagtttatgatgtgcggaagatgatcgccaaaagcgaacaagaaattggtaaagcaaccgccaaatacttcttctacagcaatattatgaacttcttcaaaaccgaaatcaccctggccaatggtgaaattcgtaaacgtccgctgatcgaaaccaatggcgaaaccggtgaaattgtttgggataaaggtcgtgattttgccaccgttcgtaaagttctgagtatgccgcaggttaacattgtgaaaaagaccgaagttcagaccggtggttttagcaaagaaagcattctgcctaaacgcaatagcgataagctgattgcccgtaaaaaagattgggacccgaaaaaatacggtggatttgatagcccgaccgttgcatatagcgttctggttgttgcaaaagtggaaaaaggtaagtccaagaaactgaaaagcgttaaagagctgctgggcattaccattatggaacgtagcagctttgaaaaaaacccgatcgatttcctggaagccaaaggttataaagaggtgaagaaagacctgattatcaagctgccaaagtatagcctgtttgaactggaaaatggtcgtaaacgcatgctggcaagtgcaggcgaactgcagaaaggtaatgaactggcactgccgagcaaatatgttaactttctgtatctggccagccactatgaaaagctgaaaggttcaccggaagataacgaacagaaacagttatttgtggaacagcacaaacactatctggatgaaattattgagcagatcagcgaatttagcaaacgtgttattctggcagatgccaatctggacaaagttctgtcagcatataacaaacaccgcgataaaccgattcgtgaacaggcagaaaacatcattcacctgtttaccctgaccaatctgggtgcaccggcagcctttaaatactttgataccaccattgatcgcaaacgttataccagcaccaaagaagttctggacgcaaccctgattcatcagagcattaccggtctgtatgaaacccgcattgatctgagccagttaggtggtgattgaagtatattttagatgaagattatttcttaatccatgggtatggacagttttccctttgatatgtaacggtgaacagttgttctacttttgtttgttagtcttgatgcttcactgatagatacaagagccataagaacctcagatccttccgtatttagccagtatgttctctagtgtggttcgttgtttttgcgtgagccatgagaacgaaccattgagatcatacttactttgcatgtcactcaaaaattttgcctcaaaactggtgagctgaatttttgcagttaaagcatcgtgtagtgtttttcttagtccgttacgtaggtaggaatctgatgtaatggttgttggtattttgtcaccattcatttttatctggttgttctcaagttcggttacgagatccatttgtctatctagttcaacttggaaaatcaacgtatcagtcgggcggcctcgcttatcaaccaccaatttcatattgctgtaagtgtttaaatctttacttattggtttcaaaacccattggttaagccttttaaactcatggtagttattttcaagcattaacatgaacttaaattcatcaaggctaatctctatatttgccttgtgagttttcttttgtgttagttcttttaataaccactcataaatcctcatagagtatttgttttcaaaagacttaacatgttccagattatattttatgaatttttttaactggaaaagataaggcaatatctcttcactaaaaactaattctaatttttcgcttgagaacttggcatagtttgtccactggaaaatctcaaagcctttaaccaaaggattcctgatttccacagttctcgtcatcagctctctggttgctttagctaatacaccataagcattttccctactgatgttcatcatctgagcgtattggttataagtgaacgataccgtccgttctttccttgtagggttttcaatcgtggggttgagtagtgccacacagcataaaattagcttggtttcatgctccgttaagtcatagcgactaatcgctagttcatttgctttgaaaacaactaattcagacatacatctcaattggtctaggtgattttaatcactataccaattgagatgggctagtcaatgataattactagtccttttcctttgagttgtgggtatctgtaaattctgctagacctttgctggaaaacttgtaaattctgctagaccctctgtaaattccgctagacctttgtgtgttttttttgtttatattcaagtggttataatttatagaataaagaaagaataaaaaaagataaaaagaatagatcccagccctgtgtataactcactactttagtcagttccgcagtattacaaaaggatgtcgcaaacgctgtttgctcctctacaaaacagaccttaaaaccctaaaggcttaagtagcaccctcgcaagctcggttgcggccgcaatcgggcaaatcgctgaatattccttttgtctccgaccatcaggcacctgagtcgctgtctttttcgtgacattcagttcgctgcgctcacggctctggcagtgaatgggggtaaatggcactacaggcgccttttatggattcatgcaaggaaactacccataatacaagaaaagcccgtcacgggcttctcagggcgttttatggcgggtctgctatgtggtgctatctgactttttgctgttcagcagttcctgccctctgattttccagtctgaccacttcggattatcccgtgacaggtcattcagactggctaatgcacccagtaaggcagcggtatcatcaacggggtctgacgctcagtggaacgaaaactcacgttaagggattttggtcatgagattatcaaaaaggatcttcacctagatccttttaaattaaaaatgaagttttaaatcaatctaaagtatatatgagtaaacttggtctgacagttaccaatgcttaatcagtgaggcacctatctcagcgatctgtctatttcgttcatccatagttgcctgactccccgtcgtgtagataactacgatacgggagggcttaccatctggccccagtgctgcaatgataccgcgagacccacgctcaccggctccagatttatcagcaataaaccagccagccggaagggccgagcgcagaagtggtcctgcaactttatccgcctccatccagtctattaattgttgccgggaagctagagtaagtagttcgccagttaatagtttgcgcaacgttgttgccattgctacaggcatcgtggtgtcacgctcgtcgtttggtatggcttcattcagctccggttcccaacgatcaaggcgagttacatgatcccccatgttgtgcaaaaaagcggttagctccttcggtcctccgatcgttgtcagaagtaagttggccgcagtgttatcactcatggttatggcagcactgcataattctcttactgtcatgccatccgtaagatgcttttctgtgactggtgagtactcaaccaagtcattctgagaatagtgtatgcggcgaccgagttgctcttgcccggcgtcaatacgggataataccgcgccacatagcagaactttaaaagtgctcatcattggaaaacgttcttcggggcgaaaactctcaaggatcttaccgctgttgagatccagttcgatgtaacccactcgtgcacccaactgatcttcagcatcttttactttcaccagcgtttctgggtgagcaaaaacaggaaggcaaaatgccgcaaaaaagggaataagggcgacacggaaatgttgaatactcatactcttcctttttcaatattattgaagcatttatcagggttattgtctcatgagcggatacatatttgaatgtatttagaaaaataaacaaataggggttccgcgcacatttccccgaaaagtgccacctgcatcgatttattatgacaacttgacggctacatcattcactttttcttcacaaccggcacggaactcgctcgggctggccccggtgcattttttaaatacccgcgagaaatagagttgatcgtcaaaaccaacattgcgaccgacggtggcgataggcatccgggtggtgctcaaaagcagcttcgcctggctgatacgttggtcctcgcgccagcttaagacgctaatccctaactgctggcggaaaagatgtgacagacgcgacggcgacaagcaaacatgctgtgcgacgctggcgatatcaaaattgctgtctgccaggtgatcgctgatgtactgacaagcctcgcgtacccgattatccatcggtggatggagcgactcgttaatcgcttccatgcgccgcagtaacaattgctcaagcagatttatcgccagcagctccgaatagcgcccttccccttgcccggcgttaatgatttgcccaaacaggtcgctgaaatgcggctggtgcgcttcatccgggcgaaagaaccccgtattggcaaatattgacggccagttaagccattcatgccagtaggcgcgcggacgaaagtaaacccactggtgataccattcgcgagcctccggatgacgaccgtagtgatgaatctctcctggcgggaacagcaaaatatcacccggtcggcaaacaaattctcgtccctgatttttcaccaccccctgaccgcgaatggtgagattgagaatataacctttcattcccagcggtcggtcgataaaaaaatcgagataaccgttggcctcaatcggcgttaaacccgccaccagatgggcattaaacgagtatcccggcagcaggggatcattttgcgcttcagccatacttttcatactcccgccattcagagaagaaaccaattgtccatattgcatcagacattgccgtcactgcgtcttttactggctcttctcgctaaccaaaccggtaaccccgcttattaaaagcattctgtaacaaagcgggaccaaagccatgacaaaaacgcgtaacaaaagtgtctataatcacggcagaaaagtccacattgattatttgcacggcgtcacactttgctatgccatagcatttttatccataagattagcggatcctacctgacgctttttatcgcaactctctactgtttctccatacccgtttttttgggaattcgagctctaaggaggttataaaaaatggatattaatactgaaactgagatcaagcaaaagcattcactaaccccctttcctgttttcctaatcagcccggcatttcgcgggcgatattttcacagctatttcaggagttcagccatgaacgcttattacattcaggatcgtcttgaggctcagagctgggcgcgtcactaccagcagctcgcccgtgaagagaaagaggcagaactggcagacgacatggaaaaaggcctgccccagcacctgtttgaatcgctatgcatcgatcatttgcaacgccacggggccagcaaaaaatccattacccgtgcgtttgatgacgatgttgagtttcaggagcgcatggcagaacacatccggtacatggttgaaaccattgctcaccaccaggttgatattgattcagaggtataaaacgaatgagtactgcactcgcaacgctggctgggaagctggctgaacgtgtcggcatggattctgtcgacccacaggaactgatcaccactcttcgccagacggcatttaaaggtgatgccagcgatgcgcagttcatcgcattactgatcgttgccaaccagtacggccttaatccgtggacgaaagaaatttacgcctttcctgataagcagaatggcatcgttccggtggtgggcgttgatggctggtcccgcatcatcaatgaaaaccagcagtttgatggcatggactttgagcaggacaatgaatcctgtacatgccggatttaccgcaaggaccgtaatcatccgatctgcgttaccgaatggatggatgaatgccgccgcgaaccattcaaaactcgcgaaggcagagaaatcacggggccgtggcagtcgcatcccaaacggatgttacgtcataaagccatgattcagtgtgcccgtctggccttcggatttgctggtatctatgacaaggatgaagccgagcgcattgtcgaaaatactgcatacactgcagaacgtcagccggaacgcgacatcactccggttaacgatgaaaccatgcaggagattaacactctgctgatcgccctggataaaacatgggatgacgacttattgccgctctgttcccagatatttcgccgcgacattcgtgcatcgtcagaactgacacaggccgaagcagtaaaagctcttggattcctgaaacagaaagccgcagagcagaaggtggcagcatgacaccggacattatcctgcagcgtaccgggatcgatgtgagagctgtcgaacagggggatgatgcgtggcacaaattacggctcggcgtcatcaccgcttcagaagttcacaacgtgatagcaaaaccccgctccggaaagaagtggcctgacatgaaaatgtcctacttccacaccctgcttgctgaggtttgcaccggtgtggctccggaagttaacgctaaagcactggcctggggaaaacagtacgagaacgacgccagaaccctgtttgaattcacttccggcgtgaatgttactgaatccccgatcatctatcgcgacgaaagtatgcgtaccgcctgctctcccgatggtttatgcagtgacggcaacggccttgaactgaaatgcccgtttacctcccgggatttcatgaagttccggctcggtggtttcgaggccataaagtcagcttacatggcccaggtgcagtacagcatgtgggtgacgcgaaaaaatgcctggtactttgccaactatgacccgcgtatgaagcgtgaaggcctgcattatgtcgtgattgagcgggatgaaaagtacatggcgagttttgacgagatcgtgccggagttcatcgaaaaaatggacgaggcactggctgaaattggttttgtatttggggagcaatggcgatgacgcatcctcacgataatatccgggtaggcgcaatcactttcgtctactccgttacaaagcgaggctgggtatttcccggcctttctgttatccgaaatccactgaaagcacagcggctggctgaggagataaataataaacgaggggctgtatgcacaaagcatcttctgttgagttaagaacgagtatcgagatggcacatagccttgctcaaattggaatcaggtttgtgccaataccagtagaaacagacgaagaatc

SEQ ID NO: 25 - DNA, 9023 bp, synthetic construct
  source 1..9023: mol_type = other DNA
ttgacaattaatcatcggctcgtataatgtgtggaattgtgagcggataacaatttcacacaggaaacagaattcaggaggcaaaaatggacaaaaaatacagcattggtctggatattggcaccaatagcgttggttgggcagttattaccgatgaatataaagttccgagcaaaaaattcaaggtgctgggtaataccgatcgccatagcattaaaaagaatctgattggtgcactgctgttcgatagcggtgaaaccgcagaagcaacccgtctgaaacgtaccgcacgtcgtcgttatacccgtcgtaaaaatcgtatttgctatctgcaagagatctttagcaacgaaatggccaaagtggatgatagcttttttcatcgtctggaagaatcctttctggtggaagaagataaaaaacacgaacgccatccgatttttggcaacattgttgatgaagtggcctaccatgaaaaatatccgaccatttatcatctgcgcaaaaaactggttgatagcaccgataaagccgatctgcgtctgatttatctggcactggcacatatgatcaaatttcgtggtcattttctgatcgaaggtgatctgaatccggataatagtgatgtggataaactgttcattcagctggtgcagacctataatcagctgtttgaagaaaatccgattaatgccagcggtgttgatgcaaaagcaattctgagcgcacgtctgagcaaaagccgtcgcctggaaaacctgattgcacagctgcctggtgaaaaaaagaatggtctgtttggtaatctgatcgcactgagcctgggtctgaccccgaactttaaatcaaattttgatctggccgaagatgccaaactgcagctgagcaaagatacctatgatgatgatctggataatctgctggcacagattggtgatcagtatgcagacctgtttctggcagcgaaaaatctgagtgatgcaattctgctgagcgatattctgcgtgttaataccgaaattaccaaagcaccgctgagcgcaagtatgattaaacgttatgatgaacatcaccaggatctgaccctgctgaaagcactggttcgtcagcagctgccggaaaagtataaagaaatctttttcgaccagagcaagaatggctatgccggttatattgatggtggtgcaagccaagaagagttctacaaattcattaaaccgatcctggaaaagatggatggcaccgaagaactgctggttaaactgaatcgtgaagatctgctgcgtaaacagcgtacctttgataatggtagcattccgcatcagattcatctgggtgaactgcatgccattctgcgtcgtcaagaagatttttatccgttcctgaaagataaccgcgagaaaatcgaaaaaattctgacctttcgcatcccgtattatgtgggtccgctggcacgtggtaatagccgttttgcatggatgacccgtaaaagcgaagaaaccattacaccgtggaatttcgaagaggttgttgataaaggtgcaagcgcacagagctttattgaacgtatgaccaacttcgataaaaacctgccgaatgaaaaagttctgccgaaacatagcctgctgtatgaatatttcaccgtgtataatgagctgaccaaagtgaaatatgtgaccgaaggtatgcgtaaaccggcatttctgagcggtgaacagaaaaaagcgattgttgatctgctgtttaaaaccaatcgtaaggttaccgttaagcagctgaaagaggattatttcaaaaaaatcgagtgctttgatagcgtcgaaattagcggtgtggaagatcgttttaatgcaagcctgggcacctatcacgatctgctgaaaatcattaaagataaagattttctggacaacgaagagaacgaggacattctggaagatattgttctgacactgaccctgtttgaggatcgtgaaatgattgaagaacgcctgaaaacatatgcccacctgttcgatgataaagtgatgaaacaactgaaacgccgtcgctataccggttggggtcgtctgagccgtaaactgattaatggtattcgtgataaacagagcggcaaaaccattctggattttctgaaaagtgatggctttgccaatcgcaattttatgcagctgattcatgatgatagcctgacctttaaagaggatattcagaaagcacaggttagcggtcagggtgatagtctgcatgaacatattgcaaatctggcaggtagtccggcaatcaaaaaaggtattctgcagaccgttaaagtggttgatgaactggttaaagttatgggtcgtcataaaccggaaaacatcgtgattgaaatggcacgtgaaaatcagaccacacagaaaggccagaaaaatagccgtgaacgcatgaaacgtattgaagaaggtattaaagaactgggcagccagattctgaaagaacatccggttgaaaatacccagctgcagaacgaaaaactgtatctgtattacctgcagaatggtcgtgacatgtatgttgatcaagaactggatattaatcgcctgagcgattatgatgtcgatcatattgttccgcagtcctttcttaaagatgatagcattgacaacaaagtgctgacccgtagcgacaaaaatcgtggtaaaagtgataatgtgccgagcgaagaggtggttaaaaagatgaaaaactattggcgtcaactgctgaacgccaaactgatcacacagcgcaaatttgataatctgacaaaagcagaacgtggtggtctgagcgagctggataaagcaggttttatcaaacgtcagctggttgaaacccgtcagatcacaaaacatgttgcacagattctggatagccgcatgaataccaaatatgacgaaaacgataaactgatccgcgaggttaaagtgattaccctgaaaagcaaactggtgagcgattttcgtaaagacttccagttttacaaagtgcgcgaaatcaacaattatcatcacgcacatgatgcctatctgaatgcagttgttggcaccgcactgattaagaaatatcctaaactggaaagcgagttcgtgtatggcgattataaagtttatgatgtgcggaagatgatcgccaaaagcgaacaagaaattggtaaagcaaccgccaaatacttcttctacagcaatattatgaacttcttcaaaaccgaaatcaccctggccaatggtgaaattcgtaaacgtccgctgatcgaaaccaatggcgaaaccggtgaaattgtttgggataaaggtcgtgattttgccaccgttcgtaaagttctgagtatgccgcaggttaacattgtgaaaaagaccgaagttcagaccggtggttttagcaaagaaagcattctgcctaaacgcaatagcgataagctgattgcccgtaaaaaagattgggacccgaaaaaatacggtggatttgatagcccgaccgttgcatatagcgttctggttgttgcaaaagtggaaaaaggtaagtccaagaaactgaaaagcgttaaagagctgctgggcattaccattatggaacgtagcagctttgaaaaaaacccgatcgatttcctggaagccaaaggttataaagaggtgaagaaagacctgattatcaagctgccaaagtatagcctgtttgaactggaaaatggtcgtaaacgcatgctggcaagtgcaggcgaactgcagaaaggtaatgaactggcactgccgagcaaatatgttaactttctgtatctggccagccactatgaaaagctgaaaggttcaccggaagataacgaacagaaacagttatttgtggaacagcacaaacactatctggatgaaattattgagcagatcagcgaatttagcaaacgtgttattctggcagatgccaatctggacaaagttctgtcagcatataacaaacaccgcgataaaccgattcgtgaacaggcagaaaacatcattcacctgtttaccctgaccaatctgggtgcaccggcagcctttaaatactttgataccaccattgatcgcaaacgttataccagcaccaaagaagttctggacgcaaccctgattcatcagagcattaccggtctgtatgaaacccgcattgatctgagccagttaggtggtgattgatgatgatgaaaaaaacgacaaagcagcactgattacagtgctgctttttttatccctgtgtggatgtggatgtggatgtggatggtaccgtggattctagaagcttggctgttttggcggatgagagaagattttcagcctgatacagattaaatcagaacgcagaagcggtctgataaaacagaatttgcctggcggcagtagcgcggtggtcccacctgaccccatgccgaactcagaagtgaaacgccgtagcgccgatggtagtgtggggtctccccatgcgagagtagggaactgccaggcatcaaataaaacgaaaggctcagtcgaaagactgggcctttcgttttatctgttgtttgtcggtgaacgctctcctgagtaggacaaatccgccgggagcggatttgaacgttgcgaagcaacggcccggagggtggcgggcaggacgcccgccataaactgccaggcatcaaattaagcagaaggccatcctgacggatggcctttttgcgtttctacaaactcttttgtttatttttctaaatacattcaaatatgtatccgctcatgagacaataaccctgataaatgcttcaataatattgaaaaaggaagagtatgagtattcaacatttccgtgtcgcccttattcccttttttgcggcattttgccttcctgtttttgctcacccagaaacgctggtgaaagtaaaagatgctgaagatcagttgggtgcacgagtgggttacatcgaactggatctcaacagcggtaagatccttgagagttttcgccccgaagaacgttttccaatgatgagcacttttgcggccgcatatgagctctccggaagatctctcgaggtcgacgtacgtgcccatggatgcatttaattaattcgaagttaacttaagcttgtacactagtaaagttctgctatgtggcgcggtattatcccgtgttgacgccgggcaagagcaactcggtcgccgcatacactattctcagaatgacttggttgagtccatggcggccgccttcatgtggcaggagaaaaaaggctgcaccggtgcgtcagcagaatatgtgatacaggatatattccgcttcctcgctcactgactcgctacgctcggtcgttcgactgcggcgagcggaaatggcttacgaacggggcggagatttcctggaagatgccaggaagatacttaacagggaagtgagagggccgcggcaaagccgtttttccataggctccgcccccctgacaagcatcacgaaatctgacgctcaaatcagtggtggcgaaacccgacaggactataaagataccaggcgtttccccctggcggctccctcgtgcgctctcctgttcctgcctttcggtttaccggtgtcattccgctgttatggccgcgtttgtctcattccacgcctgacactcagttccgggtaggcagttcgctccaagctggactgtatgcacgaaccccccgttcagtccgaccgctgcgccttatccggtaactatcgtcttgagtccaacccggaaagacatgcaaaagcaccactggcagcagccactggtaattgatttagaggagttagtcttgaagtcatgcgccggttaaggctaaactgaaaggacaagttttggtgactgcgctcctccaagccagttacctcggttcaaagagttggtagctcagagaaccttcgaaaaaccgccctgcaaggcggttttttcgttttcagagcaagagattacgcgcagaccaaaacgatctcaagaagatcatcttattaatcagataaaatatttctagctagatttcagtgcaatttatctcttcaaatgtagcacctgaagtcagccccatacgatataagttgtaattctcatgtttgacagcttatcatcgataagctccaggacccaacgctgcccgagatgcgccgcgtgcggctgctggagatggcggacgcgatggatatgttctgccaagggttggtttgcgcattcacagttctccgcaagaattgattggctccaattcttggagtggtgaatccgttagcgaggtgccgccggcttccattcaggtcgaggtggcccggctccatgcaccgcgacgcaacgcggggaggcagacaaggtatagggcggcgcctacaatccatgccaacccgttccatgtgctcgccgaggcggcataaatcgccgtgacgatcagcggtccaatgatcgaagttaggctggtaagagccgcgagcgatccttgaagctgtccctgatggtcgtcatctacctgcctggacagcatggcctgcaacgcgggcatcccgatgccgccggaagcgagaagaatcataatggggaaggccatccagcctcgcgtcgcgaacgccagcaagacgtagcccagcgcgtcggccgccatgccggcgataatggcctgcttctcgccgaaacgtttggtggcgggaccagtgacgaaggcttgagcgagggcgtgcaagattccgaataccgcaagcgacaggccgatcatcgtcgcgctccagcgaaagcggtcctcgccgaaaatgacccagagcgctgccggcacctgtcctacgagttgcatgataaagaagacagtcataagtgcggcgacgatagtcatgccccgcgcccaccggaaggagctgactgggttgaaggctctcaagggcatcggtcgacgctctcccttatgcgactcctgcattaggaagcagcccagtagtaggttgaggccgttgagcaccgccgccgcaaggaatggtgcatgcaaggagatggcgcccaacagtcccccggccacggggcctgccaccatacccacgccgaaacaagcgctcatgagcccgaagtggcgagcccgatcttccccatcggtgatgtcggcgatataggcgccagcaaccgcacctgtggcgccggtgatgccggccacgatgcgtccggcgtagaggatccacaggacgggtgtggtcgccatgatcgcgtagtcgatagtggctccaagtagcgaagcgagcaggactgggcggcggccaaagcggtcggacagtgctccgagaacgggtgcgcatagaaattgcatcaacgcatatagcgctagcagcacgccatagtgactggcgatgctgtcggaatggacgatatcccgcaagaggcccggcagtaccggcataaccaagcctatgcctacagcatccagggtgacggtgccgaggatgacgatgagcgcattgttagatttcatacacggtgcctgactgcgttagcaatttaactgtgataaactaccgcattaaagcttatcgatgataagctgtcaaacatggcctgtcgcttgcggtattcggaatcttgcacgccctcgctcaagccttcgtcactggtcccgccaccaaacgtttcggcgagaagcaggccattatcgccggcatggcggccgacgcgctgggagaggcggtttgcgtattgggcgccagggtggtttttcttttcaccagtgagacgggcaacagctgattgcccttcaccgcctggccctgagagagttgcagcaagcggtccacgctggtttgccccagcaggcgaaaatcctgtttgatggtggttaacggcgggatataacatgagctgtcttcggtatcgtcgtatcccactaccgagatatccgcaccaacgcgcagcccggactcggtaatggcgcgcattgcgcccagcgccatctgatcgttggcaaccagcatcgcagtgggaacgatgccctcattcagcatttgcatggtttgttgaaaaccggacatggcactccagtcgccttcccgttccgctatcggctgaatttgattgcgagtgagatatttatgccagccagccagacgcagacgcgccgagacagaacttaatgggcccgctaacagcgcgatttgctggtgacccaatgcgaccagatgctccacgcccagtcgcgtaccgtcttcatgggagaaaataatactgttgatgggtgtctggtcagagacatcaagaaataacgccggaacattagtgcaggcagcttccacagcaatggcatcctggtcatccagcggatagttaatgatcagcccactgacgcgttgcgcgagaagattgtgcaccgccgctttacaggcttcgacgccgcttcgttctaccatcgacaccaccacgctggcacccagttgatcggcgcgagatttaatcgccgcgacaatttgcgacggcgcgtgcagggccagactggaggtggcaacgccaatcagcaacgactgtttgcccgccagttgttgtgccacgcggttgggaatgtaattcagctccgccatcgccgcttccactttttcccgcgttttcgcagaaacgtggctggcctggttcaccacgcgggaaacggtctgataagagacaccggcatactctgcgacatcgtataacgttactggtttcacattcaccaccctgaattgactctcttccgggcgctatcatgccataccgcgaaaggttttgcaccattcgatggtgtcaacgtaaatgcatgccgcttcgccttcgcgcgcgaattgcaagctgatccgggcttatcgactgcacggtgcaccaatgcttctggcgtcaggcagccatcggaagctgtggtatggctgtgcaggtcgtaaatcactgcataattcgtgtcgctcaaggcgcactcccgttctggataatgttttttgcgccgacatcataacggttctggcaaatattgtggaattgtgagcgg

SEQ ID NO: 26 - DNA, 18 bp, synthetic construct
  source 1..18: mol_type = other DNA
catcataacggttctggc

SEQ ID NO: 27 - DNA, 20 bp, synthetic construct
  source 1..20: mol_type = other DNA
ctgcgttctgatttaatctg

SEQ ID NO: 28 - DNA, 196 bp, synthetic construct
  source 1..196: mol_type = other DNA
ttgacaattaatcatcggctcgtataatgtgtggaattgtgagcggataacaatttgttggaaccattcaaaacagcatagcaagttaaaataaggctagtccgttatcaacttgaaaaagtggcaccgagtcggtgcttttttgaaaaaaacgacaaagcagcactgattacagtgctgctttttttatccctgt

SEQ ID NO: 29 - DNA, 211 bp, synthetic construct
  source 1..211: mol_type = other DNA
ttgacaattaatcatcggctcgtataatgtgtggaattgtgagcggataacaatttgttttagagctatgctgttttgaatggtcccaaaacaaaaaaaaaaaaaaaaaaaaaaaaaaagtcgttttagagctatgctgttttgaatggtcccaaaactgaaaaaaacgacaaagcagcactgattacagtgctgctttttttatccctgt

SEQ ID NO: 30 - DNA, 32 bp, synthetic construct
  source 1..32: mol_type = other DNA
ttgcacggtaccttgacaattaatcatcggct

SEQ ID NO: 31 - DNA, 56 bp, synthetic construct
  source 1..56: mol_type = other DNA
aaattgttatccgctcacaattccacacattatacgagccgatgattaattgtcaa

SEQ ID NO: 32 - DNA, 60 bp, synthetic construct
  source 1..60: mol_type = other DNA
ttgtgagcggataacaatttgttggaaccattcaaaacagcatagcaagttaaaataagg

SEQ ID NO: 33 - DNA, 60 bp, synthetic construct
  source 1..60: mol_type = other DNA
accgactcggtgccactttttcaagttgataacggactagccttattttaacttgctatg

SEQ ID NO: 34 - DNA, 60 bp, synthetic construct
  source 1..60: mol_type = other DNA
aaaagtggcaccgagtcggtgcttttttgaaaaaaacgacaaagcagcactgattacagt

SEQ ID NO: 35 - DNA, 88 bp, synthetic construct
  source 1..88: mol_type = other DNA
ttgcactctagaatccaccccgggatccacatccacatccacatccacacagggataaaaaaagcagcactgtaatcagtgctgcttt

SEQ ID NO: 36 - DNA, 32 bp, synthetic construct
  source 1..32: mol_type = other DNA
ttgcaccccgggttgacaattaatcatcggct

SEQ ID NO: 37 - DNA, 60 bp, synthetic construct
  source 1..60: mol_type = other DNA
aaacaaattgttatccgctcacaattccacacattatacgagccgatgattaattgtcaa

SEQ ID NO: 38 - DNA, 60 bp, synthetic construct
  source 1..60: mol_type = other DNA
gagcggataacaatttgttttagagctatgctgttttgaatggtcccaaaacaaaaaaaa

SEQ ID NO: 39 - DNA, 60 bp, synthetic construct
  source 1..60: mol_type = other DNA
acagcatagctctaaaacgactttttttttttttttttttttttttttgttttgggacca

SEQ ID NO: 40 - DNA, 60 bp, synthetic construct
  source 1..60: mol_type = other DNA
tcgttttagagctatgctgttttgaatggtcccaaaactgaaaaaaacgacaaagcagca

SEQ ID NO: 41 - DNA, 63 bp, synthetic construct
  source 1..63: mol_type = other DNA
ttgcactctagaacagggataaaaaaagcagcactgtaatcagtgctgctttgtcgttttttt

SEQ ID NO: 42 - DNA, 9249 bp, synthetic construct
  source 1..9249: mol_type = other DNA
ttgacaattaatcatcggctcgtataatgtgtggaattgtgagcggataacaatttcacacaggaaacagaattcaggaggcaaaaatggacaaaaaatacagcattggtctggatattggcaccaatagcgttggttgggcagttattaccgatgaatataaagttccgagcaaaaaattcaaggtgctgggtaataccgatcgccatagcattaaaaagaatctgattggtgcactgctgttcgatagcggtgaaaccgcagaagcaacccgtctgaaacgtaccgcacgtcgtcgttatacccgtcgtaaaaatcgtatttgctatctgcaagagatctttagcaacgaaatggccaaagtggatgatagcttttttcatcgtctggaagaatcctttctggtggaagaagataaaaaacacgaacgccatccgatttttggcaacattgttgatgaagtggcctaccatgaaaaatatccgaccatttatcatctgcgcaaaaaactggttgatagcaccgataaagccgatctgcgtctgatttatctggcactggcacatatgatcaaatttcgtggtcattttctgatcgaaggtgatctgaatccggataatagtgatgtggataaactgttcattcagctggtgcagacctataatcagctgtttgaagaaaatccgattaatgccagcggtgttgatgcaaaagcaattctgagcgcacgtctgagcaaaagccgtcgcctggaaaacctgattgcacagctgcctggtgaaaaaaagaatggtctgtttggtaatctgatcgcactgagcctgggtctgaccccgaactttaaatcaaattttgatctggccgaagatgccaaactgcagctgagcaaagatacctatgatgatgatctggataatctgctggcacagattggtgatcagtatgcagacctgtttctggcagcgaaaaatctgagtgatgcaattctgctgagcgatattctgcgtgttaataccgaaattaccaaagcaccgctgagcgcaagtatgattaaacgttatgatgaacatcaccaggatctgaccctgctgaaagcactggttcgtcagcagctgccggaaaagtataaagaaatctttttcgaccagagcaagaatggctatgccggttatattgatggtggtgcaagccaagaagagttctacaaattcattaaaccgatcctggaaaagatggatggcaccgaagaactgctggttaaactgaatcgtgaagatctgctgcgtaaacagcgtacctttgataatggtagcattccgcatcagattcatctgggtgaactgcatgccattctgcgtcgtcaagaagatttttatccgttcctgaaagataaccgcgagaaaatcgaaaaaattctgacctttcgcatcccgtattatgtgggtccgctggcacgtggtaatagccgttttgcatggatgacccgtaaaagcgaagaaaccattacaccgtggaatttcgaagaggttgttgataaaggtgcaagcgcacagagctttattgaacgtatgaccaacttcgataaaaacctgccgaatgaaaaagttctgccgaaacatagcctgctgtatgaatatttcaccgtgtataatgagctgaccaaagtgaaatatgtgaccgaaggtatgcgtaaaccggcatttctgagcggtgaacagaaaaaagcgattgttgatctgctgtttaaaaccaatcgtaaggttaccgttaagcagctgaaagaggattatttcaaaaaaatcgagtgctttgatagcgtcgaaattagcggtgtggaagatcgttttaatgcaagcctgggcacctatcacgatctgctgaaaatcattaaagataaagattttctggacaacgaagagaacgaggacattctggaagatattgttctgacactgaccctgtttgaggatcgtgaaatgattgaagaacgcctgaaaacatatgcccacctgttcgatgataaagtgatgaaacaactgaaacgccgtcgctataccggttggggtcgtctgagccgtaaactgattaatggtattcgtgataaacagagcggcaaaaccattctggattttctgaaaagtgatggctttgccaatcgcaattttatgcagctgattcatgatgatagcctgacctttaaagaggatattcagaaagcacaggttagcggtcagggtgatagtctgcatgaacatattgcaaatctggcaggtagtccggcaatcaaaaaaggtattctgcagaccgttaaagtggttgatgaactggttaaagttatgggtcgtcataaaccggaaaacatcgtgattgaaatggcacgtgaaaatcagaccacacagaaaggccagaaaaatagccgtgaacgcatgaaacgtattgaagaaggtattaaagaactgggcagccagattctgaaagaacatccggttgaaaatacccagctgcagaacgaaaaactgtatctgtattacctgcagaatggtcgtgacatgtatgttgatcaagaactggatattaatcgcctgagcgattatgatgtcgatcatattgttccgcagtcctttcttaaagatgatagcattgacaacaaagtgctgacccgtagcgacaaaaatcgtggtaaaagtgataatgtgccgagcgaagaggtggttaaaaagatgaaaaactattggcgtcaactgctgaacgccaaactgatcacacagcgcaaatttgataatctgacaaaagcagaacgtggtggtctgagcgagctggataaagcaggttttatcaaacgtcagctggttgaaacccgtcagatcacaaaacatgttgcacagattctggatagccgcatgaataccaaatatgacgaaaacgataaactgatccgcgaggttaaagtgattaccctgaaaagcaaactggtgagcgattttcgtaaagacttccagttttacaaagtgcgcgaaatcaacaattatcatcacgcacatgatgcctatctgaatgcagttgttggcaccgcactgattaagaaatatcctaaactggaaagcgagttcgtgtatggcgattataaagtttatgatgtgcggaagatgatcgccaaaagcgaacaagaaattggtaaagcaaccgccaaatacttcttctacagcaatattatgaacttcttcaaaaccgaaatcaccctggccaatggtgaaattcgtaaacgtccgctgatcgaaaccaatggcgaaaccggtgaaattgtttgggataaaggtcgtgattttgccaccgttcgtaaagttctgagtatgccgcaggttaacattgtgaaaaagaccgaagttcagaccggtggttttagcaaagaaagcattctgcctaaacgcaatagcgataagctgattgcccgtaaaaaagattgggacccgaaaaaatacggtggatttgatagcccgaccgttgcatatagcgttctggttgttgcaaaagtggaaaaaggtaagtccaagaaactgaaaagcgttaaagagctgctgggcattaccattatggaacgtagcagctttgaaaaaaacccgatcgatttcctggaagccaaaggttataaagaggtgaagaaagacctgattatcaagctgccaaagtatagcctgtttgaactggaaaatggtcgtaaacgcatgctggcaagtgcaggcgaactgcagaaaggtaatgaactggcactgccgagcaaatatgttaactttctgtatctggccagccactatgaaaagctgaaaggttcaccggaagataacgaacagaaacagttatttgtggaacagcacaaacactatctggatgaaattattgagcagatcagcgaatttagcaaacgtgttattctggcagatgccaatctggacaaagttctgtcagcatataacaaacaccgcgataaaccgattcgtgaacaggcagaaaacatcattcacctgtttaccctgaccaatctgggtgcaccggcagcctttaaatactttgataccaccattgatcgcaaacgttataccagcaccaaagaagttctggacgcaaccctgattcatcagagcattaccggtctgtatgaaacccgcattgatctgagccagttaggtggtgattgatgatgatgaaaaaaacgacaaagcagcactgattacagtgctgctttttttatccctgtgtggatgtggatgtggatgtggatggtaccttgacaattaatcatcggctcgtataatgtgtggaattgtgagcggataacaatttgttggaaccattcaaaacagcatagcaagttaaaataaggctagtccgttatcaacttgaaaaagtggcaccgagtcggtgcttttttgaaaaaaacgacaaagcagcactgattacagtgctgctttttttatccctgtgtggatgtggatgtggatgtggatcccggggtggattctagaagcttggctgttttggcggatgagagaagattttcagcctgatacagattaaatcagaacgcagaagcggtctgataaaacagaatttgcctggcggcagtagcgcggtggtcccacctgaccccatgccgaactcagaagtgaaacgccgtagcgccgatggtagtgtggggtctccccatgcgagagtagggaactgccaggcatcaaataaaacgaaaggctcagtcgaaagactgggcctttcgttttatctgttgtttgtcggtgaacgctctcctgagtaggacaaatccgccgggagcggatttgaacgttgcgaagcaacggcccggagggtggcgggcaggacgcccgccataaactgccaggcatcaaattaagcagaaggccatcctgacggatggcctttttgcgtttctacaaactcttttgtttatttttctaaatacattcaaatatgtatccgctcatgagacaataaccctgataaatgcttcaataatattgaaaaaggaagagtatgagtattcaacatttccgtgtcgcccttattcccttttttgcggcattttgccttcctgtttttgctcacccagaaacgctggtgaaagtaaaagatgctgaagatcagttgggtgcacgagtgggttacatcgaactggatctcaacagcggtaagatccttgagagttttcgccccgaagaacgttttccaatgatgagcacttttgcggccgcatatgagctctccggaagatctctcgaggtcgacgtacgtgcccatggatgcatttaattaattcgaagttaacttaagcttgtacactagtaaagttctgctatgtggcgcggtattatcccgtgttgacgccgggcaagagcaactcggtcgccgcatacactattctcagaatgacttggttgagtccatggcggccgccttcatgtggcaggagaaaaaaggctgcaccggtgcgtcagcagaatatgtgatacaggatatattccgcttcctcgctcactgactcgctacgctcggtcgttcgactgcggcgagcggaaatggcttacgaacggggcggagatttcctggaagatgccaggaagatacttaacagggaagtgagagggccgcggcaaagccgtttttccataggctccgcccccctgacaagcatcacgaaatctgacgctcaaatcagtggtggcgaaacccgacaggactataaagataccaggcgtttccccctggcggctccctcgtgcgctctcctgttcctgcctttcggtttaccggtgtcattccgctgttatggccgcgtttgtctcattccacgcctgacactcagttccgggtaggcagttcgctccaagctggactgtatgcacgaaccccccgttcagtccgaccgctgcgccttatccggtaactatcgtcttgagtccaacccggaaagacatgcaaaagcaccactggcagcagccactggtaattgatttagaggagttagtcttgaagtcatgcgccggttaaggctaaactgaaaggacaagttttggtgactgcgctcctccaagccagttacctcggttcaaagagttggtagctcagagaaccttcgaaaaaccgccctgcaaggcggttttttcgttttcagagcaagagattacgcgcagaccaaaacgatctcaagaagatcatcttattaatcagataaaatatttctagctagatttcagtgcaatttatctcttcaaatgtagcacctgaagtcagccccatacgatataagttgtaattctcatgtttgacagcttatcatcgataagctccaggacccaacgctgcccgagatgcgccgcgtgcggctgctggagatggcggacgcgatggatatgttctgccaagggttggtttgcgcattcacagttctccgcaagaattgattggctccaattcttggagtggtgaatccgttagcgaggtgccgccggcttccattcaggtcgaggtggcccggctccatgcaccgcgacgcaacgcggggaggcagacaaggtatagggcggcgcctacaatccatgccaacccgttccatgtgctcgccgaggcggcataaatcgccgtgacgatcagcggtccaatgatcgaagttaggctggtaagagccgcgagcgatccttgaagctgtccctgatggtcgtcatctacctgcctggacagcatggcctgcaacgcgggcatcccgatgccgccggaagcgagaagaatcataatggggaaggccatccagcctcgcgtcgcgaacgccagcaagacgtagcccagcgcgtcggccgccatgccggcgataatggcctgcttctcgccgaaacgtttggtggcgggaccagtgacgaaggcttgagcgagggcgtgcaagattccgaataccgcaagcgacaggccgatcatcgtcgcgctccagcgaaagcggtcctcgccgaaaatgacccagagcgctgccggcacctgtcctacgagttgcatgataaagaagacagtcataagtgcggcgacgatagtcatgccccgcgcccaccggaaggagctgactgggttgaaggctctcaagggcatcggtcgacgctctcccttatgcgactcctgcattaggaagcagcccagtagtaggttgaggccgttgagcaccgccgccgcaaggaatggtgcatgcaaggagatggcgcccaacagtcccccggccacggggcctgccaccatacccacgccgaaacaagcgctcatgagcccgaagtggcgagcccgatcttccccatcggtgatgtcggcgatataggcgccagcaaccgcacctgtggcgccggtgatgccggccacgatgcgtccggcgtagaggatccacaggacgggtgtggtcgccatgatcgcgtagtcgatagtggctccaagtagcgaagcgagcaggactgggcggcggccaaagcggtcggacagtgctccgagaacgggtgcgcatagaaattgcatcaacgcatatagcgctagcagcacgccatagtgactggcgatgctgtcggaatggacgatatcccgcaagaggcccggcagtaccggcataaccaagcctatgcctacagcatccagggtgacggtgccgaggatgacgatgagcgcattgttagatttcatacacggtgcctgactgcgttagcaatttaactgtgataaactaccgcattaaagcttatcgatgataagctgtcaaacatggcctgtcgcttgcggtattcggaatcttgcacgccctcgctcaagccttcgtcactggtcccgccaccaaacgtttcggcgagaagcaggccattatcgccggcatggcggccgacgcgctgggagaggcggtttgcgtattgggcgccagggtggtttttcttttcaccagtgagacgggcaacagctgattgcccttcaccgcctggccctgagagagttgcagcaagcggtccacgctggtttgccccagcaggcgaaaatcctgtttgatggtggttaacggcgggatataacatgagctgtcttcggtatcgtcgtatcccactaccgagatatccgcaccaacgcgcagcccggactcggtaatggcgcgcattgcgcccagcgccatctgatcgttggcaaccagcatcgcagtgggaacgatgccctcattcagcatttgcatggtttgttgaaaaccggacatggcactccagtcgccttcccgttccgctatcggctgaatttgattgcgagtgagatatttatgccagccagccagacgcagacgcgccgagacagaacttaatgggcccgctaacagcgcgatttgctggtgacccaatgcgaccagatgctccacgcccagtcgcgtaccgtcttcatgggagaaaataatactgttgatgggtgtctggtcagagacatcaagaaataacgccggaacattagtgcaggcagcttccacagcaatggcatcctggtcatccagcggatagttaatgatcagcccactgacgcgttgcgcgagaagattgtgcaccgccgctttacaggcttcgacgccgcttcgttctaccatcgacaccaccacgctggcacccagttgatcggcgcgagatttaatcgccgcgacaatttgcgacggcgcgtgcagggccagactggaggtggcaacgccaatcagcaacgactgtttgcccgccagttgttgtgccacgcggttgggaatgtaattcagctccgccatcgccgcttccactttttcccgcgttttcgcagaaacgtggctggcctggttcaccacgcgggaaacggtctgataagagacaccggcatactctgcgacatcgtataacgttactggtttcacattcaccaccctgaattgactctcttccgggcgctatcatgccataccgcgaaaggttttgcaccattcgatggtgtcaacgtaaatgcatgccgcttcgccttcgcgcgcgaattgcaagctgatccgggcttatcgactgcacggtgcaccaatgcttctggcgtcaggcagccatcggaagctgtggtatggctgtgcaggtcgtaaatcactgcataattcgtgtcgctcaaggcgcactcccgttctggataatgttttttgcgccgacatcataacggttctggcaaatattgtggaattgtgagcgg

SEQ ID NO: 43 - DNA, 9454 bp, synthetic construct
  source 1..9454: mol_type = other DNA
ttgacaattaatcatcggctcgtataatgtgtggaattgtgagcggataacaatttcacacaggaaacagaattcaggaggcaaaaatggacaaaaaatacagcattggtctggatattggcaccaatagcgttggttgggcagttattaccgatgaatataaagttccgagcaaaaaattcaaggtgctgggtaataccgatcgccatagcattaaaaagaatctgattggtgcactgctgttcgatagcggtgaaaccgcagaagcaacccgtctgaaacgtaccgcacgtcgtcgttatacccgtcgtaaaaatcgtatttgctatctgcaagagatctttagcaacgaaatggccaaagtggatgatagcttttttcatcgtctggaagaatcctttctggtggaagaagataaaaaacacgaacgccatccgatttttggcaacattgttgatgaagtggcctaccatgaaaaatatccgaccatttatcatctgcgcaaaaaactggttgatagcaccgataaagccgatctgcgtctgatttatctggcactggcacatatgatcaaatttcgtggtcattttctgatcgaaggtgatctgaatccggataatagtgatgtggataaactgttcattcagctggtgcagacctataatcagctgtttgaagaaaatccgattaatgccagcggtgttgatgcaaaagcaattctgagcgcacgtctgagcaaaagccgtcgcctggaaaacctgattgcacagctgcctggtgaaaaaaagaatggtctgtttggtaatctgatcgcactgagcctgggtctgaccccgaactttaaatcaaattttgatctggccgaagatgccaaactgcagctgagcaaagatacctatgatgatgatctggataatctgctggcacagattggtgatcagtatgcagacctgtttctggcagcgaaaaatctgagtgatgcaattctgctgagcgatattctgcgtgttaataccgaaattaccaaagcaccgctgagcgcaagtatgattaaacgttatgatgaacatcaccaggatctgaccctgctgaaagcactggttcgtcagcagctgccggaaaagtataaagaaatctttttcgaccagagcaagaatggctatgccggttatattgatggtggtgcaagccaagaagagttctacaaattcattaaaccgatcctggaaaagatggatggcaccgaagaactgctggttaaactgaatcgtgaagatctgctgcgtaaacagcgtacctttgataatggtagcattccgcatcagattcatctgggtgaactgcatgccattctgcgtcgtcaagaagatttttatccgttcctgaaagataaccgcgagaaaatcgaaaaaattctgacctttcgcatcccgtattatgtgggtccgctggcacgtggtaatagccgttttgcatggatgacccgtaaaagcgaagaaaccattacaccgtggaatttcgaagaggttgttgataaaggtgcaagcgcacagagctttattgaacgtatgaccaacttcgataaaaacctgccgaatgaaaaagttctgccgaaacatagcctgctgtatgaatatttcaccgtgtataatgagctgaccaaagtgaaatatgtgaccgaaggtatgcgtaaaccggcatttctgagcggtgaacagaaaaaagcgattgttgatctgctgtttaaaaccaatcgtaaggttaccgttaagcagctgaaagaggattatttcaaaaaaatcgagtgctttgatagcgtcgaaattagcggtgtggaagatcgttttaatgcaagcctgggcacctatcacgatctgctgaaaatcattaaagataaagattttctggacaacgaagagaacgaggacattctggaagatattgttctgacactgaccctgtttgaggatcgtgaaatgattgaagaacgcctgaaaacatatgcccacctgttcgatgataaagtgatgaaacaactgaaacgccgtcgctataccggttggggtcgtctgagccgtaaactgattaatggtattcgtgataaacagagcggcaaaaccattctggattttctgaaaagtgatggctttgccaatcgcaattttatgcagctgattcatgatgatagcctgacctttaaagaggatattcagaaagcacaggttagcggtcagggtgatagtctgcatgaacatattgcaaatctggcaggtagtccggcaatcaaaaaaggtattctgcagaccgttaaagtggttgatgaactggttaaagttatgggtcgtcataaaccggaaaacatcgtgattgaaatggcacgtgaaaatcagaccacacagaaaggccagaaaaatagccgtgaacgcatgaaacgtattgaagaaggtattaaagaactgggcagccagattctgaaagaacatccggttgaaaatacccagctgcagaacgaaaaactgtatctgtattacctgcagaatggtcgtgacatgtatgttgatcaagaactggatattaatcgcctgagcgattatgatgtcgatcatattgttccgcagtcctttcttaaagatgatagcattgacaacaaagtgctgacccgtagcgacaaaaatcgtggtaaaagtgataatgtgccgagcgaagaggtggttaaaaagatgaaaaactattggcgtcaactgctgaacgccaaactgatcacacagcgcaaatttgataatctgacaaaagcagaacgtggtggtctgagcgagctggataaagcaggttttatcaaacgtcagctggttgaaacccgtcagatcacaaaacatgttgcacagattctggatagccgcatgaataccaaatatgacgaaaacgataaactgatccgcgaggttaaagtgattaccctgaaaagcaaactggtgagcgattttcgtaaagacttccagttttacaaagtgcgcgaaatcaacaattatcatcacgcacatgatgcctatctgaatgcagttgttggcaccgcactgattaagaaatatcctaaactggaaagcgagttcgtgtatggcgattataaagtttatgatgtgcggaagatgatcgccaaaagcgaacaagaaattggtaaagcaaccgccaaatacttcttctacagcaatattatgaacttcttcaaaaccgaaatcaccctggccaatggtgaaattcgtaaacgtccgctgatcgaaaccaatggcgaaaccggtgaaattgtttgggataaaggtcgtgattttgccaccgttcgtaaagttctgagtatgccgcaggttaacattgtgaaaaagaccgaagttcagaccggtggttttagcaaagaaagcattctgcctaaacgcaatagcgataagctgattgcccgtaaaaaagattgggacccgaaaaaatacggtggatttgatagcccgaccgttgcatatagcgttctggttgttgcaaaagtggaaaaaggtaagtccaagaaactgaaaagcgttaaagagctgctgggcattaccattatggaacgtagcagctttgaaaaaaacccgatcgatttcctggaagccaaaggttataaagaggtgaagaaagacctgattatcaagctgccaaagtatagcctgtttgaactggaaaatggtcgtaaacgcatgctggcaagtgcaggcgaactgcagaaaggtaatgaactggcactgccgagcaaatatgttaactttctgtatctggccagccactatgaaaagctgaaaggttcaccggaagataacgaacagaaacagttatttgtggaacagcacaaacactatctggatgaaattattgagcagatcagcgaatttagcaaacgtgttattctggcagatgccaatctggacaaagttctgtcagcatataacaaacaccgcgataaaccgattcgtgaacaggcagaaaacatcattcacctgtttaccctgaccaatctgggtgcaccggcagcctttaaatactttgataccaccattgatcgcaaacgttataccagcaccaaagaagttctggacgcaaccctgattcatcagagcattaccggtctgtatgaaacccgcattgatctgagccagttaggtggtgattgatgatgatgaaaaaaacgacaaagcagcactgattacagtgctgctttttttatccctgtgtggatgtggatgtggatgtggatggtaccttgacaattaatcatcggctcgtataatgtgtggaattgtgagcggataacaatttgttggaaccattcaaaacagcatagcaagttaaaataaggctagtccgttatcaacttgaaaaagtggcaccgagtcggtgcttttttgaaaaaaacgacaaagcagcactgattacagtgctgctttttttatccctgtgtggatgtggatgtggatgtggatcccgggttgacaattaatcatcggctcgtataatgtgtggaattgtgagcggataacaatttgttttagagctatgctgttttgaatggtcccaaaacaaaaaaaaaaaaaaaaaaaaaaaaaaagtcgttttagagctatgctgttttgaatggtcccaaaactgaaaaaaacgacaaagcagcactgattacagtgctgctttttttatccctgttctagaagcttggctgttttggcggatgagagaagattttcagcctgatacagattaaatcagaacgcagaagcggtctgataaaacagaatttgcctggcggcagtagcgcggtggtcccacctgaccccatgccgaactcagaagtgaaacgccgtagcgccgatggtagtgtggggtctccccatgcgagagtagggaactgccaggcatcaaataaaacgaaaggctcagtcgaaagactgggcctttcgttttatctgttgtttgtcggtgaacgctctcctgagtaggacaaatccgccgggagcggatttgaacgttgcgaagcaacggcccggagggtggcgggcaggacgcccgccataaactgccaggcatcaaattaagcagaaggccatcctgacggatggcctttttgcgtttctacaaactcttttgtttatttttctaaatacattcaaatatgtatccgctcatgagacaataaccctgataaatgcttcaataatattgaaaaaggaagagtatgagtattcaacatttccgtgtcgcccttattcccttttttgcggcattttgccttcctgtttttgctcacccagaaacgctggtgaaagtaaaagatgctgaagatcagttgggtgcacgagtgggttacatcgaactggatctcaacagcggtaagatccttgagagttttcgccccgaagaacgttttccaatgatgagcacttttgcggccgcatatgagctctccggaagatctctcgaggtcgacgtacgtgcccatggatgcatttaattaattcgaagttaacttaagcttgtacactagtaaagttctgctatgtggcgcggtattatcccgtgttgacgccgggcaagagcaactcggtcgccgcatacactattctcagaatgacttggttgagtccatggcggccgccttcatgtggcaggagaaaaaaggctgcaccggtgcgtcagcagaatatgtgatacaggatatattccgcttcctcgctcactgactcgctacgctcggtcgttcgactgcggcgagcggaaatggcttacgaacggggcggagatttcctggaagatgccaggaagatacttaacagggaagtgagagggccgcggcaaagccgtttttccataggctccgcccccctgacaagcatcacgaaatctgacgctcaaatcagtggtggcgaaacccgacaggactataaagataccaggcgtttccccctggcggctccctcgtgcgctctcctgttcctgcctttcggtttaccggtgtcattccgctgttatggccgcgtttgtctcattccacgcctgacactcagttccgggtaggcagttcgctccaagctggactgtatgcacgaaccccccgttcagtccgaccgctgcgccttatccggtaactatcgtcttgagtccaacccggaaagacatgcaaaagcaccactggcagcagccactggtaattgatttagaggagttagtcttgaagtcatgcgccggttaaggctaaactgaaaggacaagttttggtgactgcgctcctccaagccagttacctcggttcaaagagttggtagctcagagaaccttcgaaaaaccgccctgcaaggcggttttttcgttttcagagcaagagattacgcgcagaccaaaacgatctcaagaagatcatcttattaatcagataaaatatttctagctagatttcagtgcaatttatctcttcaaatgtagcacctgaagtcagccccatacgatataagttgtaattctcatgtttgacagcttatcatcgataagctccaggacccaacgctgcccgagatgcgccgcgtgcggctgctggagatggcggacgcgatggatatgttctgccaagggttggtttgcgcattcacagttctccgcaagaattgattggctccaattcttggagtggtgaatccgttagcgaggtgccgccggcttccattcaggtcgaggtggcccggctccatgcaccgcgacgcaacgcggggaggcagacaaggtatagggcggcgcctacaatccatgccaacccgttccatgtgctcgccgaggcggcataaatcgccgtgacgatcagcggtccaatgatcgaagttaggctggtaagagccgcgagcgatccttgaagctgtccctgatggtcgtcatctacctgcctggacagcatggcctgcaacgcgggcatcccgatgccgccggaagcgagaagaatcataatggggaaggccatccagcctcgcgtcgcgaacgccagcaagacgtagcccagcgcgtcggccgccatgccggcgataatggcctgcttctcgccgaaacgtttggtggcgggaccagtgacgaaggcttgagcgagggcgtgcaagattccgaataccgcaagcgacaggccgatcatcgtcgcgctccagcgaaagcggtcctcgccgaaaatgacccagagcgctgccggcacctgtcctacgagttgcatgataaagaagacagtcataagtgcggcgacgatagtcatgccccgcgcccaccggaaggagctgactgggttgaaggctctcaagggcatcggtcgacgctctcccttatgcgactcctgcattaggaagcagcccagtagtaggttgaggccgttgagcaccgccgccgcaaggaatggtgcatgcaaggagatggcgcccaacagtcccccggccacggggcctgccaccatacccacgccgaaacaagcgctcatgagcccgaagtggcgagcccgatcttccccatcggtgatgtcggcgatataggcgccagcaaccgcacctgtggcgccggtgatgccggccacgatgcgtccggcgtagaggatccacaggacgggtgtggtcgccatgatcgcgtagtcgatagtggctccaagtagcgaagcgagcaggactgggcggcggccaaagcggtcggacagtgctccgagaacgggtgcgcatagaaattgcatcaacgcatatagcgctagcagcacgccatagtgactggcgatgctgtcggaatggacgatatcccgcaagaggcccggcagtaccggcataaccaagcctatgcctacagcatccagggtgacggtgccgaggatgacgatgagcgcattgttagatttcatacacggtgcctgactgcgttagcaatttaactgtgataaactaccgcattaaagcttatcgatgataagctgtcaaacatggcctgtcgcttgcggtattcggaatcttgcacgccctcgctcaagccttcgtcactggtcccgccaccaaacgtttcggcgagaagcaggccattatcgccggcatggcggccgacgcgctgggagaggcggtttgcgtattgggcgccagggtggtttttcttttcaccagtgagacgggcaacagctgattgcccttcaccgcctggccctgagagagttgcagcaagcggtccacgctggtttgccccagcaggcgaaaatcctgtttgatggtggttaacggcgggatataacatgagctgtcttcggtatcgtcgtatcccactaccgagatatccgcaccaacgcgcagcccggactcggtaatggcgcgcattgcgcccagcgccatctgatcgttggcaaccagcatcgcagtgggaacgatgccctcattcagcatttgcatggtttgttgaaaaccggacatggcactccagtcgccttcccgttccgctatcggctgaatttgattgcgagtgagatatttatgccagccagccagacgcagacgcgccgagacagaacttaatgggcccgctaacagcgcgatttgctggtgacccaatgcgaccagatgctccacgcccagtcgcgtaccgtcttcatgggagaaaataatactgttgatgggtgtctggtcagagacatcaagaaataacgccggaacattagtgcaggcagcttccacagcaatggcatcctggtcatccagcggatagttaatgatcagcccactgacgcgttgcgcgagaagattgtgcaccgccgctttacaggcttcgacgccgcttcgttctaccatcgacaccaccacgctggcacccagttgatcggcgcgagatttaatcgccgcgacaatttgcgacggcgcgtgcagggccagactggaggtggcaacgccaatcagcaacgactgtttgcccgccagttgttgtgccacgcggttgggaatgtaattcagctccgccatcgccgcttccactttttcccgcgttttcgcagaaacgtggctggcctggttcaccacgcgggaaacggtctgataagagacaccggcatactctgcgacatcgtataacgttactggtttcacattcaccaccctgaattgactctcttccgggcgctatcatgccataccgcgaaaggttttgcaccattcgatggtgtcaacgtaaatgcatgccgcttcgccttcgcgcgcgaattgcaagctgatccgggcttatcgactgcacggtgcaccaatgcttctggcgtcaggcagccatcggaagctgtggtatggctgtgcaggtcgtaaatcactgcataattcgtgtcgctcaaggcgcactcccgttctggataatgttttttgcgccgacatcataacggttctggcaaatattgtggaattgtgagcgg

SEQ ID NO: 44 - DNA, 7922 bp, synthetic construct
  source 1..7922: mol_type = other DNA
ctcgagataacgtggctttttttggtaagcagaaaataagtcattagtgaaaatatgtgtaggctggagctgcttcgaagttcctatactttctagagaataggaacttcggaataggaacttcaagatccccttattagaagaactcgtcaagaaggcgatagaaggcgatgcgctgcgaatcgggagcggcgataccgtaaagcacgaggaagcggtcagcccattcgccgccaagctcttcagcaatatcacgggtagccaacgctatgtcctgatagcggtccgccacacccagccggccacagtcgatgaatccagaaaagcggccattttccaccatgatattcggcaagcaggcatcgccatgggtcacgacgagatcctcgccgtcgggcatgcgcgccttgagcctggcgaacagttcggctggcgcgagcccctgatgctcttcgtccagatcatcctgatcgacaagaccggcttccatccgagtacgtgctcgctcgatgcgatgtttcgcttggtggtcgaatgggcaggtagccggatcaagcgtatgcagccgccgcattgcatcagccatgatggatactttctcggcaggagcaaggtgagatgacaggagatcctgccccggcacttcgcccaatagcagccagtcccttcccgcttcagtgacaacgtcgagcacagctgcgcaaggaacgcccgtcgtggccagccacgatagccgcgctgcctcgtcctgcagttcattcagggcaccggacaggtcggtcttgacaaaaagaaccgggcgcccctgcgctgacagccggaacacggcggcatcagagcagccgattgtctgttgtgcccagtcatagccgaatagcctctccacccaagcggccggagaacctgcgtgcaatccatcttgttcaatcatgcgaaacgatcctcatcctgtctcttgatcagatcttgatcccctgcgccatcagatccttggcggcaagaaagccatccagtttactttgcagggcttcccaaccttaccagagggcgccccagctggcaattccggttcgcttgctgtccataaaaccgcccagtctagctatcgccatgtaagcccactgcaagctacctgctttctctttgcgcttgcgttttcccttgtccagatagcccagtagctgacattcatccggggtcagcaccgtttctgcggactggctttctacgtgttccgcttcctttagcagcccttgcgccctgagtgcttgcggcagcgtgagcttcaaaagcgctctgaagttcctatactttctagagaataggaacttcgaactgcaggtcgacggatccccggaattaattctcatgtttgacagagaggcggtttgcgtattgggcgccagggtggtttttcttttcaccagtgagacgggcaacagctgattgcccttcaccgcctggccctgagagagttgcagcaagcggtccacgctggtttgccccagcaggcgaaaatcctgtttgatggtggttaacggcgggatataacatgagctgtcttcggtatcgtcgtatcccactaccgagatatccgcaccaacgcgcagcccggactcggtaatggcgcgcattgcgcccagcgccatctgatcgttggcaaccagcatcgcagtgggaacgatgccctcattcagcatttgcatggtttgttgaaaaccggacatggcactccagtcgccttcccgttccgctatcggctgaatttgattgcgagtgagatatttatgccagccagccagacgcagacgcgccgagacagaacttaatgggcccgctaacagcgcgatttgctggtgacccaatgcgaccagatgctccacgcccagtcgcgtaccgtcttcatgggagaaaataatactgttgatgggtgtctggtcagagacatcaagaaataacgccggaacattagtgcaggcagcttccacagcaatggcatcctggtcatccagcggatagttaatgatcagcccactgacgcgttgcgcgagaagattgtgcaccgccgctttacaggcttcgacgccgcttcgttctaccatcgacaccaccacgctggcacccagttgatcggcgcgagatttaatcgccgcgacaatttgcgacggcgcgtgcagggccagactggaggtggcaacgccaatcagcaacgactgtttgcccgccagttgttgtgccacgcggttgggaatgtaattcagctccgccatcgccgcttccactttttcccgcgttttcgcagaaacgtggctggcctggttcaccacgcgggaaacggtctgataagagacaccggcatactctgcgacatcgtataacgttactggtttcacattcaccaccctgaattgactctcttccgggcgctatcatgccataccgcgaaaggttttgcaccattcgatggtgtcaacgtaaatgcatgccgcttcgccttcgcgcgcgaattgcaagctgatccgggcttatcgactgcacggtgcaccaatgcttctggcgtcaggcagccatcggaagctgtggtatggctgtgcaggtcgtaaatcactgcataattcgtgtcgctcaaggcgcactcccgttctggataatgttttttgcgccgacatcataacggttctggcaaatattgtggaattgtgagcggttgacaattaatcatcggctcgtataatgtgtggaattgtgagcggataacaatttcacacaggaaacagaattcaggaggcaaaaatggacaaaaaatacagcattggtctggatattggcaccaatagcgttggttgggcagttattaccgatgaatataaagttccgagcaaaaaattcaaggtgctgggtaataccgatcgccatagcattaaaaagaatctgattggtgcactgctgttcgatagcggtgaaaccgcagaagcaacccgtctgaaacgtaccgcacgtcgtcgttatacccgtcgtaaaaatcgtatttgctatctgcaagagatctttagcaacgaaatggccaaagtggatgatagcttttttcatcgtctggaagaatcctttctggtggaagaagataaaaaacacgaacgccatccgatttttggcaacattgttgatgaagtggcctaccatgaaaaatatccgaccatttatcatctgcgcaaaaaactggttgatagcaccgataaagccgatctgcgtctgatttatctggcactggcacatatgatcaaatttcgtggtcattttctgatcgaaggtgatctgaatccggataatagtgatgtggataaactgttcattcagctggtgcagacctataatcagctgtttgaagaaaatccgattaatgccagcggtgttgatgcaaaagcaattctgagcgcacgtctgagcaaaagccgtcgcctggaaaacctgattgcacagctgcctggtgaaaaaaagaatggtctgtttggtaatctgatcgcactgagcctgggtctgaccccgaactttaaatcaaattttgatctggccgaagatgccaaactgcagctgagcaaagatacctatgatgatgatctggataatctgctggcacagattggtgatcagtatgcagacctgtttctggcagcgaaaaatctgagtgatgcaattctgctgagcgatattctgcgtgttaataccgaaattaccaaagcaccgctgagcgcaagtatgattaaacgttatgatgaacatcaccaggatctgaccctgctgaaagcactggttcgtcagcagctgccggaaaagtataaagaaatctttttcgaccagagcaagaatggctatgccggttatattgatggtggtgcaagccaagaagagttctacaaattcattaaaccgatcctggaaaagatggatggcaccgaagaactgctggttaaactgaatcgtgaagatctgctgcgtaaacagcgtacctttgataatggtagcattccgcatcagattcatctgggtgaactgcatgccattctgcgtcgtcaagaagatttttatccgttcctgaaagataaccgcgagaaaatcgaaaaaattctgacctttcgcatcccgtattatgtgggtccgctggcacgtggtaatagccgttttgcatggatgacccgtaaaagcgaagaaaccattacaccgtggaatttcgaagaggttgttgataaaggtgcaagcgcacagagctttattgaacgtatgaccaacttcgataaaaacctgccgaatgaaaaagttctgccgaaacatagcctgctgtatgaatatttcaccgtgtataatgagctgaccaaagtgaaatatgtgaccgaaggtatgcgtaaaccggcatttctgagcggtgaacagaaaaaagcgattgttgatctgctgtttaaaaccaatcgtaaggttaccgttaagcagctgaaagaggattatttcaaaaaaatcgagtgctttgatagcgtcgaaattagcggtgtggaagatcgttttaatgcaagcctgggcacctatcacgatctgctgaaaatcattaaagataaagattttctggacaacgaagagaacgaggacattctggaagatattgttctgacactgaccctgtttgaggatcgtgaaatgattgaagaacgcctgaaaacatatgcccacctgttcgatgataaagtgatgaaacaactgaaacgccgtcgctataccggttggggtcgtctgagccgtaaactgattaatggtattcgtgataaacagagcggcaaaaccattctggattttctgaaaagtgatggctttgccaatcgcaattttatgcagctgattcatgatgatagcctgacctttaaagaggatattcagaaagcacaggttagcggtcagggtgatagtctgcatgaacatattgcaaatctggcaggtagtccggcaatcaaaaaaggtattctgcagaccgttaaagtggttgatgaactggttaaagttatgggtcgtcataaaccggaaaacatcgtgattgaaatggcacgtgaaaatcagaccacacagaaaggccagaaaaatagccgtgaacgcatgaaacgtattgaagaaggtattaaagaactgggcagccagattctgaaagaacatccggttgaaaatacccagctgcagaacgaaaaactgtatctgtattacctgcagaatggtcgtgacatgtatgttgatcaagaactggatattaatcgcctgagcgattatgatgtcgatcatattgttccgcagtcctttcttaaagatgatagcattgacaacaaagtgctgacccgtagcgacaaaaatcgtggtaaaagtgataatgtgccgagcgaagaggtggttaaaaagatgaaaaactattggcgtcaactgctgaacgccaaactgatcacacagcgcaaatttgataatctgacaaaagcagaacgtggtggtctgagcgagctggataaagcaggttttatcaaacgtcagctggttgaaacccgtcagatcacaaaacatgttgcacagattctggatagccgcatgaataccaaatatgacgaaaacgataaactgatccgcgaggttaaagtgattaccctgaaaagcaaactggtgagcgattttcgtaaagacttccagttttacaaagtgcgcgaaatcaacaattatcatcacgcacatgatgcctatctgaatgcagttgttggcaccgcactgattaagaaatatcctaaactggaaagcgagttcgtgtatggcgattataaagtttatgatgtgcggaagatgatcgccaaaagcgaacaagaaattggtaaagcaaccgccaaatacttcttctacagcaatattatgaacttcttcaaaaccgaaatcaccctggccaatggtgaaattcgtaaacgtccgctgatcgaaaccaatggcgaaaccggtgaaattgtttgggataaaggtcgtgattttgccaccgttcgtaaagttctgagtatgccgcaggttaacattgtgaaaaagaccgaagttcagaccggtggttttagcaaagaaagcattctgcctaaacgcaatagcgataagctgattgcccgtaaaaaagattgggacccgaaaaaatacggtggatttgatagcccgaccgttgcatatagcgttctggttgttgcaaaagtggaaaaaggtaagtccaagaaactgaaaagcgttaaagagctgctgggcattaccattatggaacgtagcagctttgaaaaaaacccgatcgatttcctggaagccaaaggttataaagaggtgaagaaagacctgattatcaagctgccaaagtatagcctgtttgaactggaaaatggtcgtaaacgcatgctggcaagtgcaggcgaactgcagaaaggtaatgaactggcactgccgagcaaatatgttaactttctgtatctggccagccactatgaaaagctgaaaggttcaccggaagataacgaacagaaacagttatttgtggaacagcacaaacactatctggatgaaattattgagcagatcagcgaatttagcaaacgtgttattctggcagatgccaatctggacaaagttctgtcagcatataacaaacaccgcgataaaccgattcgtgaacaggcagaaaacatcattcacctgtttaccctgaccaatctgggtgcaccggcagcctttaaatactttgataccaccattgatcgcaaacgttataccagcaccaaagaagttctggacgcaaccctgattcatcagagcattaccggtctgtatgaaacccgcattgatctgagccagttaggtggtgattgatgatgatgaaaaaaacgacaaagcagcactgattacagtgctgctttttttatccctgtgtggatgtggatgtggatgtggatggtaccttgacaattaatcatcggctcgtataatgtgtggaattgtgagcggataacaatttgttggaaccattcaaaacagcatagcaagttaaaataaggctagtccgttatcaacttgaaaaagtggcaccgagtcggtgcttttttgaaaaaaacgacaaagcagcactgattacagtgctgctttttttatccctgtgtggatgtggatgtggatgtggatcccgggttgacaattaatcatcggctcgtataatgtgtggaattgtgagcggataacaatttgttttagagctatgctgttttgaatggtcccaaaacaaaaaaaaaaaaaaaaaaaaaaaaaaagtcgttttagagctatgctgttttgaatggtcccaaaactgaaaaaaacgacaaagcagcactgattacagtgctgctttttttatccctgttctagaagcttggctgttttggcggatgagagaagattttcagcctgatacagattaaatcagaacgcagaagcggtctgataaaacagaatttgcctggcggcagtagcgcggtggtcccacctgaccccatgccgaactcagaagtgaaacgccgtagcgccgatggtagtgtggggtctccccatgcgagagtagggaactgccaggcatcaaataaaacgaaaggctcagtcgaaagactgggcctttcgttttatctgttgtttgtcggtgaacgctctcctgagtaggacaaatccgccgggagcggatttgaacgttgcgaagcaacggcccggagggtggcgggcaggacgcccgccataaactgccaggcatcaaattaagcagaaggccatcctgacggatggcctttttgcgtttctacaaactctttacttattgtttgaaatcacgggggcgcaccgtataatttgaccgctttttgctcgag

SEQ ID NO: 45 - DNA, 18 bp, synthetic construct
  source 1..18: mol_type = other DNA
tccgcttcctttagcagc

SEQ ID NO: 46 - DNA, 18 bp, synthetic construct
  source 1..18: mol_type = other DNA
gctttacaggcttcgacg

SEQ ID NO: 47 - DNA, 18 bp, synthetic construct
  source 1..18: mol_type = other DNA
gctgggtaataccgatcg

SEQ ID NO: 48 - DNA, 20 bp, synthetic construct
  source 1..20: mol_type = other DNA
aattaccaaagcaccgctga

SEQ ID NO: 49 - DNA, 20 bp, synthetic construct
  source 1..20: mol_type = other DNA
cacctatcacgatctgctga

SEQ ID NO: 50 - DNA, 18 bp, synthetic construct
  source 1..18: mol_type = other DNA
gagcgaagaggtggttaa

SEQ ID NO: 51 - DNA, 20 bp, synthetic construct
  source 1..20: mol_type = other DNA
tgttgcaaaagtggaaaaag

SEQ ID NO: 52 - DNA, 20 bp, synthetic construct
  source 1..20: mol_type = other DNA
taatgtgtggaattgtgagc

SEQ ID NO: 53 - DNA, 18 bp, synthetic construct
  source 1..18: mol_type = other DNA
ggtgaacgctctcctgag

SEQ ID NO: 54 - DNA, 22 bp, synthetic construct
  source 1..22: mol_type = other DNA
ggttagactgttaacaacaacc

SEQ ID NO: 55 - DNA, 21 bp, synthetic construct
  source 1..21: mol_type = other DNA
catcacgtttttcactcctgc